European Patent Specification EP 3 415 531 B1, published September 6, 2023. Title: Antigen Binding Proteins. Applicant: CRAIGEN, Jennifer WATTAM, Trevor Anthony Kenneth PARMER, Radha Shah MAYES, Patrick HAMBLIN, Paul Andrew CLEGG, Stephanie ALGATE, Paul LEWIS, Alan Peter. The sequence listing filed with the application follows.

SEQUENCE LISTING (199 sequences)

SEQ ID NO: 1 - protein, 5 aa, mus musculus
NYWMH

SEQ ID NO: 2 - protein, 17 aa, mus musculus
ATYRGHSDTYYNQKFKG

SEQ ID NO: 3 - protein, 12 aa, mus musculus
GAIYNGYDVLDN

SEQ ID NO: 4 - protein, 11 aa, mus musculus
SASQDISNYLN

SEQ ID NO: 5 - protein, 7 aa, mus musculus
YTSNLHS

SEQ ID NO: 6 - protein, 9 aa, mus musculus
QQYRKLPWT

SEQ ID NO: 7 - protein, 121 aa, mus musculus
EVQLQQSGAVLARPGASVKMSCKGSGYTFTNYWMHWVKQRPGQGLEWIGATYRGHSDTYYNQKFKGKAKLTAVTSTSTAYMELSSLTNEDSAVYYCTRGAIYNGYDVLDNWGQGTLVTVSS

SEQ ID NO: 8 - DNA, 363 bp, mus musculus
gaggtgcagctgcagcagagcggcgccgtgctggccaggcccggagctagcgtgaagatgagctgcaagggcagcggctacaccttcaccaactactggatgcactgggtgaaacagaggcccggccagggactggagtggatcggcgccacctacaggggccacagcgacacctactacaaccagaagttcaagggcaaggccaagctgaccgccgtgacctcaaccagcaccgcctacatggaactgagcagcctgaccaacgaggacagcgccgtctattactgcaccaggggcgccatctacaacggctacgacgtgctggacaattggggccagggaacactagtgaccgtgtccagc

SEQ ID NO: 9 - protein, 108 aa, mus musculus
DIQLTQTTSSLSASLGDRVTISCSASQDISNYLNWYQQKPDGTVELVIYYTSNLHSGVPSRFSGSGSGTDYSLTIGYLEPEDVATYYCQQYRKLPWTFGGGSKLEIKR

SEQ ID NO: 10 - DNA, 324 bp, mus musculus
gatatccagctgacccagaccacaagcagcctgagcgcctccctgggcgacagggtgaccattagctgcagcgccagccaggacatcagcaactacctgaactggtaccagcagaagcccgacggcaccgtggagctcgtgatctactacacctccaacctgcacagcggcgtgcccagcaggttctctggcagcggcagcggcaccgactacagcctgaccatcggctatctggagcccgaggacgtcgccacctactactgccagcagtacaggaagctgccctggaccttcggcggaggctctaagctggagattaagcgt

SEQ ID NO: 11 - protein, 121 aa, Artificial Sequence
  Humansed antibody sequence
QVQLVQSGAEVKKPGSSVKVSCKASGGTFSNYWMHWVRQAPGQGLEWMGATYRGHSDTYYNQKFKGRVTITADKSTSTAYMELSSLRSEDTAVYYCARGAIYNGYDVLDNWGQGTLVTVSS

SEQ ID NO: 12 - DNA, 363 bp, Artificial Sequence
  Humansed antibody sequence
caggtgcagctggtccagagcggcgccgaagtgaagaagcccggcagctccgtgaaagtgagctgcaaggccagcggcggcaccttcagcaactactggatgcactgggtgaggcaggcccccggacagggcctggagtggatgggcgccacctacaggggccacagcgacacctactacaaccagaagttcaagggccgggtgaccatcaccgccgacaagagcaccagcaccgcctacatggaactgagcagcctcaggagcgaggacaccgctgtgtattactgcgccaggggcgccatctacaacggctacgacgtgctggacaactggggccagggcacactagtgaccgtgtccagc

SEQ ID NO: 13 - protein, 121 aa, Artificial Sequence
  Humansed antibody sequence
QVQLVQSGAEVKKPGSSVKVSCKASGYTFTNYWMHWVRQAPGQGLEWMGATYRGHSDTYYNQKFKGRVTITADKSTSTAYMELSSLRSEDTAVYYCARGAIYNGYDVLDNWGQGTLVTVSS

SEQ ID NO: 14 - DNA, 363 bp, Artificial Sequence
  Humansed antibody sequence
caggtgcagctggtccagagcggcgccgaagtgaagaagcccggcagctccgtgaaagtgagctgcaaggccagcggctacaccttcaccaactactggatgcactgggtgaggcaggcccccggacagggcctggagtggatgggcgccacctacaggggccacagcgacacctactacaaccagaagttcaagggccgggtgaccatcaccgccgacaagagcaccagcaccgcctacatggaactgagcagcctcaggagcgaggacaccgctgtgtattactgcgccaggggcgccatctacaacggctacgacgtgctggacaactggggccagggcacactagtgaccgtgtccagc

SEQ ID NO: 15 - protein, 121 aa, Artificial Sequence
  Humansed antibody sequence
QVQLVQSGAEVKKPGSSVKVSCKASGYTFTNYWMHWVRQAPGQGLEWMGATYRGHSDTYYNQKFKGRVTITADKSTSTAYMELSSLRSEDTAVYYCTRGAIYNGYDVLDNWGQGTLVTVSS

SEQ ID NO: 16 - DNA, 363 bp, Artificial Sequence
  Humansed antibody sequence
caggtgcagctggtccagagcggcgccgaagtgaagaagcccggcagctccgtgaaagtgagctgcaaggccagcggctacaccttcaccaactactggatgcactgggtgaggcaggcccccggacagggcctggagtggatgggcgccacctacaggggccacagcgacacctactacaaccagaagttcaagggccgggtgaccatcaccgccgacaagagcaccagcaccgcctacatggaactgagcagcctcaggagcgaggacaccgctgtgtattactgcaccaggggcgccatctacaacggctacgacgtgctggacaactggggccagggcacactagtgaccgtgtccagc

SEQ ID NO: 17 - protein, 121 aa, Artificial Sequence
  Humansed antibody sequence
QVQLVQSGAEVKKPGSSVKVSCKGSGYTFTNYWMHWVRQAPGQGLEWMGATYRGHSDTYYNQKFKGRVTITADTSTSTAYMELSSLRSEDTAVYYCTRGAIYNGYDVLDNWGQGTLVTVSS

SEQ ID NO: 18 - DNA, 363 bp, Artificial Sequence
  Humansed antibody sequence
caggtgcagctggtccagagcggcgccgaagtgaagaagcccggcagctccgtgaaagtgagctgcaagggcagcggctacaccttcaccaactactggatgcactgggtgaggcaggcccccggacagggcctggagtggatgggcgccacctacaggggccacagcgacacctactacaaccagaagttcaagggccgggtgaccatcaccgccgacacgagcaccagcaccgcctacatggaactgagcagcctcaggagcgaggacaccgctgtgtattactgcaccaggggcgccatctacaacggctacgacgtgctggacaactggggccagggcacactagtgaccgtgtccagc

SEQ ID NO: 19 - protein, 121 aa, Artificial Sequence
  Humansed antibody sequence
QVQLVQSGAEVKKPGSSVKVSCKGSGYTFTNYWMHWVRQAPGQGLEWIGATYRGHSDTYYNQKFKGRATLTADTSTSTAYMELSSLRSEDTAVYYCTRGAIYNGYDVLDNWGQGTLVTVSS

SEQ ID NO: 20 - DNA, 363 bp, Artificial Sequence
  Humansed antibody sequence
caggtgcagctggtccagagcggcgccgaagtgaagaagcccggcagctccgtgaaagtgagctgcaagggcagcggctacaccttcaccaactactggatgcactgggtgaggcaggcccccggacagggcctggagtggatcggcgccacctacaggggccacagcgacacctactacaaccagaagttcaagggccgggcgaccctcaccgccgacacgagcaccagcaccgcctacatggaactgagcagcctcaggagcgaggacaccgctgtgtattactgcaccaggggcgccatctacaacggctacgacgtgctggacaactggggccagggcacactagtgaccgtgtccagc

SEQ ID NO: 21 - protein, 121 aa, Artificial Sequence
  Humansed antibody sequence
QVQLVQSGAEVKKPGSSVKVSCKGSGYTFTNYWMHWVRQAPGQGLEWMGATYRGHSDTYYNQKFKGRVTITADTSTSTAYMELSSLRSEDTAVYYCTRGAIYDGYDVLDNWGQGTLVTVSS

SEQ ID NO: 22 - DNA, 363 bp, Artificial Sequence
  Humansed antibody sequence
caggtgcagctggtccagagcggcgccgaagtgaagaagcccggcagctccgtgaaagtgagctgcaagggcagcggctacaccttcaccaactactggatgcactgggtgaggcaggcccccggacagggcctggagtggatgggcgccacctacaggggccacagcgacacctactacaaccagaagttcaagggccgggtgaccatcaccgccgacacgagcaccagcaccgcctacatggaactgagcagcctcaggagcgaggacaccgctgtgtattactgcaccaggggcgccatctacgacggctacgacgtgctggacaactggggccagggcacactagtgaccgtgtccagc

SEQ ID NO: 23 - protein, 121 aa, Artificial Sequence
  Humansed antibody sequence
QVQLVQSGAEVKKPGSSVKVSCKASGGTFSNYWMHWVRQAPGQGLEWMGATYRGHSDTYYNQKFKGRVTITADKSTSTAYMELSSLRSEDTAVYYCARGAIYDGYDVLDNWGQGTLVTVSS

SEQ ID NO: 24 - DNA, 363 bp, Artificial Sequence
  Humansed antibody sequence
caggtgcagctggtccagagcggcgccgaagtgaagaagcccggcagctccgtgaaagtgagctgcaaggccagcggcggcaccttcagcaactactggatgcactgggtgaggcaggcccccggacagggcctggagtggatgggcgccacctacaggggccacagcgacacctactacaaccagaagttcaagggccgggtgaccatcaccgccgacaagagcaccagcaccgcctacatggaactgagcagcctcaggagcgaggacaccgctgtgtattactgcgccaggggcgccatctacgacggctacgacgtgctggacaactggggccagggcacactagtgaccgtgtccagc

SEQ ID NO: 25 - protein, 121 aa, Artificial Sequence
  Humansed antibody sequence
QVQLVQSGAEVKKPGSSVKVSCKASGYTFTNYWMHWVRQAPGQGLEWMGATYRGHSDTYYNQKFKGRVTITADKSTSTAYMELSSLRSEDTAVYYCARGAIYDGYDVLDNWGQGTLVTVSS

SEQ ID NO: 26 - DNA, 363 bp, Artificial Sequence
  Humansed antibody sequence
caggtgcagctggtccagagcggcgccgaagtgaagaagcccggcagctccgtgaaagtgagctgcaaggccagcggctacaccttcaccaactactggatgcactgggtgaggcaggcccccggacagggcctggagtggatgggcgccacctacaggggccacagcgacacctactacaaccagaagttcaagggccgggtgaccatcaccgccgacaagagcaccagcaccgcctacatggaactgagcagcctcaggagcgaggacaccgctgtgtattactgcgccaggggcgccatctacgacggctacgacgtgctggacaactggggccagggcacactagtgaccgtgtccagc

SEQ ID NO: 27 - protein, 121 aa, Artificial Sequence
  Humansed antibody sequence
QVQLVQSGAEVKKPGSSVKVSCKASGYTFTNYWMHWVRQAPGQGLEWMGATYRGHSDTYYNQKFKGRVTITADKSTSTAYMELSSLRSEDTAVYYCTRGAIYDGYDVLDNWGQGTLVTVSS

SEQ ID NO: 28 - DNA, 363 bp, Artificial Sequence
  Humansed antibody sequence
caggtgcagctggtccagagcggcgccgaagtgaagaagcccggcagctccgtgaaagtgagctgcaaggccagcggctacaccttcaccaactactggatgcactgggtgaggcaggcccccggacagggcctggagtggatgggcgccacctacaggggccacagcgacacctactacaaccagaagttcaagggccgggtgaccatcaccgccgacaagagcaccagcaccgcctacatggaactgagcagcctcaggagcgaggacaccgctgtgtattactgcaccaggggcgccatctacgacggctacgacgtgctggacaactggggccagggcacactagtgaccgtgtccagc

SEQ ID NO: 29 - protein, 121 aa, Artificial Sequence
  Humansed antibody sequence
QVQLVQSGAEVKKPGSSVKVSCKGSGYTFTNYWMHWVRQAPGQGLEWIGATYRGHSDTYYNQKFKGRATLTADTSTSTAYMELSSLRSEDTAVYYCTRGAIYDGYDVLDNWGQGTLVTVSS

SEQ ID NO: 30 - DNA, 363 bp, Artificial Sequence
  Humansed antibody sequence
caggtgcagctggtccagagcggcgccgaagtgaagaagcccggcagctccgtgaaagtgagctgcaagggcagcggctacaccttcaccaactactggatgcactgggtgaggcaggcccccggacagggcctggagtggatcggcgccacctacaggggccacagcgacacctactacaaccagaagttcaagggccgggcgaccctcaccgccgacacgagcaccagcaccgcctacatggaactgagcagcctcaggagcgaggacaccgctgtgtattactgcaccaggggcgccatctacgacggctacgacgtgctggacaactggggccagggcacactagtgaccgtgtccagc

SEQ ID NO: 31 - protein, 108 aa, Artificial Sequence
  Humansed antibody sequence
DIQMTQSPSSLSASVGDRVTITCSASQDISNYLNWYQQKPGKAPKLLIYYTSNLHSGVPSRFSGSGSGTDFTLTISSLQPEDFATYYCQQYRKLPWTFGQGTKLEIKR

SEQ ID NO: 32 - DNA, 324 bp, Artificial Sequence
  Humansed antibody sequence
gacatccagatgacccagagccctagctcactgagcgccagcgtgggcgacagggtgaccattacctgctccgccagccaggacatcagcaactacctgaactggtaccagcagaagcccggcaaggcccccaagctgctgatctactacacctccaacctgcactccggcgtgcccagcaggttcagcggaagcggcagcggcaccgatttcaccctgaccatctccagcctgcagcccgaggacttcgccacctactactgccagcagtacaggaagctcccctggactttcggccagggcaccaaactggagatcaagcgt

SEQ ID NO: 33 - protein, 108 aa, Artificial Sequence
  Humansed antibody sequence
DIQMTQSPSSLSASVGDRVTITCSASQDISNYLNWYQQKPGKAPKLLIYYTSNLHSGVPSRFSGSGSGTDYTLTISSLQPEDFATYYCQQYRKLPWTFGQGTKLEIKR

SEQ ID NO: 34 - DNA, 324 bp, Artificial Sequence
  Humansed antibody sequence
gacatccagatgacccagagccctagctcactgagcgccagcgtgggcgacagggtgaccattacctgctccgccagccaggacatcagcaactacctgaactggtaccagcagaagcccggcaaggcccccaagctgctgatctactacacctccaacctgcactccggcgtgcccagcaggttcagcggaagcggcagcggcaccgattacaccctgaccatctccagcctgcagcccgaggacttcgccacctactactgccagcagtacaggaagctcccctggactttcggccagggcaccaaactggagatcaagcgt

SEQ ID NO: 35 - protein, 108 aa, Artificial Sequence
  Humansed antibody sequence
DIQLTQSPSSLSASVGDRVTITCSASQDISNYLNWYQQKPGKAPELVIYYTSNLHSGVPSRFSGSGSGTDYTLTISSLQPEDFATYYCQQYRKLPWTFGQGTKLEIKR

SEQ ID NO: 36 - DNA, 324 bp, Artificial Sequence
  Humansed antibody sequence
gacatccagctgacccagagccctagctcactgagcgccagcgtgggcgacagggtgaccattacctgctccgccagccaggacatcagcaactacctgaactggtaccagcagaagcccggcaaggcccccgagctggtgatctactacacctccaacctgcactccggcgtgcccagcaggttcagcggaagcggcagcggcaccgattacaccctgaccatctccagcctgcagcccgaggacttcgccacctactactgccagcagtacaggaagctcccctggactttcggccagggcaccaaactggagatcaagcgt

SEQ ID NO: 37 - protein, 310 aa, homo sapiens
MPLLLLLPLLWAGALAMLQMAGQCSQNEYFDSLLHACIPCQLRCSSNTPPLTCQRYCNASVTNSVKGTNSGENLYFQGDPKSCDKTHTCPPCPAPELLGGPSVFLFPPKPKDTLMISRTPEVTCVVVDVSHEDPEVKFNWYVDGVEVHNAKTKPREEQYNSTYRVVSVLTVLHQDWLNGKEYKCKVSNKALPAPIEKTISKAKGQPREPQVYTLPPSRDELTKNQVSLTCLVKGFYPSDIAVEWESNGQPENNYKTTPPVLDSDGSFFLYSKLTVDKSRWQQGNVFSCSVMHEALHNHYTQKSLSLSPGK

SEQ ID NO: 38 - DNA, 930 bp, homo sapiens
atgccgctgctgctactgctgcccctgctgtgggcaggggcgctagctatgctgcagatggccggccagtgcagccagaacgagtacttcgacagcctgctgcacgcctgcatcccctgccagctgagatgcagcagcaacacacctcctctgacctgccagagatactgcaacgccagcgtgaccaacagcgtgaagggcaccaactccggagagaacctgtacttccaaggggatcccaaatcttgtgacaaaactcacacatgcccaccgtgcccagcacctgaactcctggggggaccgtcagtcttcctcttccccccaaaacccaaggacaccctcatgatctcccggacccctgaggtcacatgcgtggtggtggacgtgagccacgaagaccctgaggtcaagttcaactggtacgtggacggcgtggaggtgcataatgccaagacaaagccgcgggaggagcagtacaacagcacgtaccgtgtggtcagcgtcctcaccgtcctgcaccaggactggctgaatggcaaggagtacaagtgcaaggtctccaacaaagccctcccagcccccatcgagaaaaccatctccaaagccaaagggcagccccgagagccacaggtgtacaccctgcccccatcccgggatgagctgaccaagaaccaggtcagcctgacctgcctggtcaaaggcttctatcccagcgacatcgccgtggagtgggagagcaatgggcagccggagaacaactacaagaccacgcctcccgtgctggactccgacggctccttcttcctctacagcaagctcaccgtggacaagagcaggtggcagcaggggaacgtcttctcatgctccgtgatgcatgaggctctgcacaaccactacacgcagaagagcctctccctgtctccgggtaaa

SEQ ID NO: 39 - protein, 307 aa, homo sapiens
MPLLLLLPLLWAGALAMAGQCSQNEYFDSLLHACIPCQLRCSSNTPPLTCQRYCNASVTNSVKGTNSGENLYFQGDPKSCDKTHTCPPCPAPELLGGPSVFLFPPKPKDTLMISRTPEVTCVVVDVSHEDPEVKFNWYVDGVEVHNAKTKPREEQYNSTYRVVSVLTVLHQDWLNGKEYKCKVSNKALPAPIEKTISKAKGQPREPQVYTLPPSRDELTKNQVSLTCLVKGFYPSDIAVEWESNGQPENNYKTTPPVLDSDGSFFLYSKLTVDKSRWQQGNVFSCSVMHEALHNHYTQKSLSLSPGK

SEQ ID NO: 40 - DNA, 921 bp, homo sapiens
atgccgctgctgctactgctgcccctgctgtgggcaggggcgctagctatggccggccagtgcagccagaacgagtacttcgacagcctgctgcacgcctgcatcccctgccagctgagatgcagcagcaacacacctcctctgacctgccagagatactgcaacgccagcgtgaccaacagcgtgaagggcaccaactccggagagaacctgtacttccaaggggatcccaaatcttgtgacaaaactcacacatgcccaccgtgcccagcacctgaactcctggggggaccgtcagtcttcctcttccccccaaaacccaaggacaccctcatgatctcccggacccctgaggtcacatgcgtggtggtggacgtgagccacgaagaccctgaggtcaagttcaactggtacgtggacggcgtggaggtgcataatgccaagacaaagccgcgggaggagcagtacaacagcacgtaccgtgtggtcagcgtcctcaccgtcctgcaccaggactggctgaatggcaaggagtacaagtgcaaggtctccaacaaagccctcccagcccccatcgagaaaaccatctccaaagccaaagggcagccccgagagccacaggtgtacaccctgcccccatcccgggatgagctgaccaagaaccaggtcagcctgacctgcctggtcaaaggcttctatcccagcgacatcgccgtggagtgggagagcaatgggcagccggagaacaactacaagaccacgcctcccgtgctggactccgacggctccttcttcctctacagcaagctcaccgtggacaagagcaggtggcagcaggggaacgtcttctcatgctccgtgatgcatgaggctctgcacaaccactacacgcagaagagcctctccctgtctccgggtaaa

SEQ ID NO: 41 - protein, 306 aa, cynomolgous macaque
MPLLLLLPLLWAGALAMARQCSQNEYFDSLLHDCKPCQLRCSSTPPLTCQRYCNASMTNSVKGMNSGENLYFQGDPKSCDKTHTCPPCPAPELLGGPSVFLFPPKPKDTLMISRTPEVTCVVVDVSHEDPEVKFNWYVDGVEVHNAKTKPREEQYNSTYRVVSVLTVLHQDWLNGKEYKCKVSNKALPAPIEKTISKAKGQPREPQVYTLPPSRDELTKNQVSLTCLVKGFYPSDIAVEWESNGQPENNYKTTPPVLDSDGSFFLYSKLTVDKSRWQQGNVFSCSVMHEALHNHYTQKSLSLSPGK

SEQ ID NO: 42 - DNA, 918 bp, cynomolgous macaque
atgccgctgctgctactgctgcccctgctgtgggcaggggcgctagctatggccagacagtgcagccagaacgagtacttcgacagcctgctgcacgactgcaagccctgccagctgagatgcagcagcacacctcctctgacctgccagagatactgcaacgccagcatgaccaacagcgtgaagggcatgaactccggagagaacctgtacttccaaggggatcccaaatcttgtgacaaaactcacacatgcccaccgtgcccagcacctgaactcctggggggaccgtcagtcttcctcttccccccaaaacccaaggacaccctcatgatctcccggacccctgaggtcacatgcgtggtggtggacgtgagccacgaagaccctgaggtcaagttcaactggtacgtggacggcgtggaggtgcataatgccaagacaaagccgcgggaggagcagtacaacagcacgtaccgtgtggtcagcgtcctcaccgtcctgcaccaggactggctgaatggcaaggagtacaagtgcaaggtctccaacaaagccctcccagcccccatcgagaaaaccatctccaaagccaaagggcagccccgagagccacaggtgtacaccctgcccccatcccgggatgagctgaccaagaaccaggtcagcctgacctgcctggtcaaaggcttctatcccagcgacatcgccgtggagtgggagagcaatgggcagccggagaacaactacaagaccacgcctcccgtgctggactccgacggctccttcttcctctacagcaagctcaccgtggacaagagcaggtggcagcaggggaacgtcttctcatgctccgtgatgcatgaggctctgcacaaccactacacgcagaagagcctctccctgtctccgggtaaa

SEQ ID NO: 43 - protein, 451 aa, Artificial Sequence
  Humansed antibody sequence
QVQLVQSGAEVKKPGSSVKVSCKASGGTFSNYWMHWVRQAPGQGLEWMGATYRGHSDTYYNQKFKGRVTITADKSTSTAYMELSSLRSEDTAVYYCARGAIYNGYDVLDNWGQGTLVTVSSASTKGPSVFPLAPSSKSTSGGTAALGCLVKDYFPEPVTVSWNSGALTSGVHTFPAVLQSSGLYSLSSVVTVPSSSLGTQTYICNVNHKPSNTKVDKKVEPKSCDKTHTCPPCPAPELLGGPSVFLFPPKPKDTLMISRTPEVTCVVVDVSHEDPEVKFNWYVDGVEVHNAKTKPREEQYNSTYRVVSVLTVLHQDWLNGKEYKCKVSNKALPAPIEKTISKAKGQPREPQVYTLPPSRDELTKNQVSLTCLVKGFYPSDIAVEWESNGQPENNYKTTPPVLDSDGSFFLYSKLTVDKSRWQQGNVFSCSVMHEALHNHYTQKSLSLSPGK

SEQ ID NO: 44 - DNA, 1353 bp, Artificial Sequence
  Humansed antibody sequence
caggtgcagctggtccagagcggcgccgaagtgaagaagcccggcagctccgtgaaagtgagctgcaaggccagcggcggcaccttcagcaactactggatgcactgggtgaggcaggcccccggacagggcctggagtggatgggcgccacctacaggggccacagcgacacctactacaaccagaagttcaagggccgggtgaccatcaccgccgacaagagcaccagcaccgcctacatggaactgagcagcctcaggagcgaggacaccgctgtgtattactgcgccaggggcgccatctacaacggctacgacgtgctggacaactggggccagggcacactagtgaccgtgtccagcgccagcaccaagggccccagcgtgttccccctggcccccagcagcaagagcaccagcggcggcacagccgccctgggctgcctggtgaaggactacttccccgaaccggtgaccgtgtcctggaacagcggagccctgaccagcggcgtgcacaccttccccgccgtgctgcagagcagcggcctgtacagcctgagcagcgtggtgaccgtgcccagcagcagcctgggcacccagacctacatctgtaacgtgaaccacaagcccagcaacaccaaggtggacaagaaggtggagcccaagagctgtgacaagacccacacctgccccccctgccctgcccccgagctgctgggaggccccagcgtgttcctgttcccccccaagcctaaggacaccctgatgatcagcagaacccccgaggtgacctgtgtggtggtggatgtgagccacgaggaccctgaggtgaagttcaactggtacgtggacggcgtggaggtgcacaatgccaagaccaagcccagggaggagcagtacaacagcacctaccgggtggtgtccgtgctgaccgtgctgcaccaggattggctgaacggcaaggagtacaagtgtaaggtgtccaacaaggccctgcctgcccctatcgagaaaaccatcagcaaggccaagggccagcccagagagccccaggtgtacaccctgccccctagcagagatgagctgaccaagaaccaggtgtccctgacctgcctggtgaagggcttctaccccagcgacatcgccgtggagtgggagagcaacggccagcccgagaacaactacaagaccaccccccctgtgctggacagcgatggcagcttcttcctgtacagcaagctgaccgtggacaagagcagatggcagcagggcaacgtgttcagctgctccgtgatgcacgaggccctgcacaatcactacacccagaagagcctgagcctgtcccctggcaag

SEQ ID NO: 45 - protein, 451 aa, Artificial Sequence
  Humansed antibody sequence
QVQLVQSGAEVKKPGSSVKVSCKASGYTFTNYWMHWVRQAPGQGLEWMGATYRGHSDTYYNQKFKGRVTITADKSTSTAYMELSSLRSEDTAVYYCARGAIYNGYDVLDNWGQGTLVTVSSASTKGPSVFPLAPSSKSTSGGTAALGCLVKDYFPEPVTVSWNSGALTSGVHTFPAVLQSSGLYSLSSVVTVPSSSLGTQTYICNVNHKPSNTKVDKKVEPKSCDKTHTCPPCPAPELLGGPSVFLFPPKPKDTLMISRTPEVTCVVVDVSHEDPEVKFNWYVDGVEVHNAKTKPREEQYNSTYRVVSVLTVLHQDWLNGKEYKCKVSNKALPAPIEKTISKAKGQPREPQVYTLPPSRDELTKNQVSLTCLVKGFYPSDIAVEWESNGQPENNYKTTPPVLDSDGSFFLYSKLTVDKSRWQQGNVFSCSVMHEALHNHYTQKSLSLSPGK

SEQ ID NO: 46 - DNA, 1353 bp, Artificial Sequence
  Humansed antibody sequence
caggtgcagctggtccagagcggcgccgaagtgaagaagcccggcagctccgtgaaagtgagctgcaaggccagcggctacaccttcaccaactactggatgcactgggtgaggcaggcccccggacagggcctggagtggatgggcgccacctacaggggccacagcgacacctactacaaccagaagttcaagggccgggtgaccatcaccgccgacaagagcaccagcaccgcctacatggaactgagcagcctcaggagcgaggacaccgctgtgtattactgcgccaggggcgccatctacaacggctacgacgtgctggacaactggggccagggcacactagtgaccgtgtccagcgccagcaccaagggccccagcgtgttccccctggcccccagcagcaagagcaccagcggcggcacagccgccctgggctgcctggtgaaggactacttccccgaaccggtgaccgtgtcctggaacagcggagccctgaccagcggcgtgcacaccttccccgccgtgctgcagagcagcggcctgtacagcctgagcagcgtggtgaccgtgcccagcagcagcctgggcacccagacctacatctgtaacgtgaaccacaagcccagcaacaccaaggtggacaagaaggtggagcccaagagctgtgacaagacccacacctgccccccctgccctgcccccgagctgctgggaggccccagcgtgttcctgttcccccccaagcctaaggacaccctgatgatcagcagaacccccgaggtgacctgtgtggtggtggatgtgagccacgaggaccctgaggtgaagttcaactggtacgtggacggcgtggaggtgcacaatgccaagaccaagcccagggaggagcagtacaacagcacctaccgggtggtgtccgtgctgaccgtgctgcaccaggattggctgaacggcaaggagtacaagtgtaaggtgtccaacaaggccctgcctgcccctatcgagaaaaccatcagcaaggccaagggccagcccagagagccccaggtgtacaccctgccccctagcagagatgagctgaccaagaaccaggtgtccctgacctgcctggtgaagggcttctaccccagcgacatcgccgtggagtgggagagcaacggccagcccgagaacaactacaagaccaccccccctgtgctggacagcgatggcagcttcttcctgtacagcaagctgaccgtggacaagagcagatggcagcagggcaacgtgttcagctgctccgtgatgcacgaggccctgcacaatcactacacccagaagagcctgagcctgtcccctggcaag

SEQ ID NO: 47 - protein, 451 aa, Artificial Sequence
  Humansed antibody sequence
QVQLVQSGAEVKKPGSSVKVSCKASGYTFTNYWMHWVRQAPGQGLEWMGATYRGHSDTYYNQKFKGRVTITADKSTSTAYMELSSLRSEDTAVYYCTRGAIYNGYDVLDNWGQGTLVTVSSASTKGPSVFPLAPSSKSTSGGTAALGCLVKDYFPEPVTVSWNSGALTSGVHTFPAVLQSSGLYSLSSVVTVPSSSLGTQTYICNVNHKPSNTKVDKKVEPKSCDKTHTCPPCPAPELLGGPSVFLFPPKPKDTLMISRTPEVTCVVVDVSHEDPEVKFNWYVDGVEVHNAKTKPREEQYNSTYRVVSVLTVLHQDWLNGKEYKCKVSNKALPAPIEKTISKAKGQPREPQVYTLPPSRDELTKNQVSLTCLVKGFYPSDIAVEWESNGQPENNYKTTPPVLDSDGSFFLYSKLTVDKSRWQQGNVFSCSVMHEALHNHYTQKSLSLSPGK

SEQ ID NO: 48 - DNA, 1353 bp, Artificial Sequence
  Humansed antibody sequence
caggtgcagctggtccagagcggcgccgaagtgaagaagcccggcagctccgtgaaagtgagctgcaaggccagcggctacaccttcaccaactactggatgcactgggtgaggcaggcccccggacagggcctggagtggatgggcgccacctacaggggccacagcgacacctactacaaccagaagttcaagggccgggtgaccatcaccgccgacaagagcaccagcaccgcctacatggaactgagcagcctcaggagcgaggacaccgctgtgtattactgcaccaggggcgccatctacaacggctacgacgtgctggacaactggggccagggcacactagtgaccgtgtccagcgccagcaccaagggccccagcgtgttccccctggcccccagcagcaagagcaccagcggcggcacagccgccctgggctgcctggtgaaggactacttccccgaaccggtgaccgtgtcctggaacagcggagccctgaccagcggcgtgcacaccttccccgccgtgctgcagagcagcggcctgtacagcctgagcagcgtggtgaccgtgcccagcagcagcctgggcacccagacctacatctgtaacgtgaaccacaagcccagcaacaccaaggtggacaagaaggtggagcccaagagctgtgacaagacccacacctgccccccctgccctgcccccgagctgctgggaggccccagcgtgttcctgttcccccccaagcctaaggacaccctgatgatcagcagaacccccgaggtgacctgtgtggtggtggatgtgagccacgaggaccctgaggtgaagttcaactggtacgtggacggcgtggaggtgcacaatgccaagaccaagcccagggaggagcagtacaacagcacctaccgggtggtgtccgtgctgaccgtgctgcaccaggattggctgaacggcaaggagtacaagtgtaaggtgtccaacaaggccctgcctgcccctatcgagaaaaccatcagcaaggccaagggccagcccagagagccccaggtgtacaccctgccccctagcagagatgagctgaccaagaaccaggtgtccctgacctgcctggtgaagggcttctaccccagcgacatcgccgtggagtgggagagcaacggccagcccgagaacaactacaagaccaccccccctgtgctggacagcgatggcagcttcttcctgtacagcaagctgaccgtggacaagagcagatggcagcagggcaacgtgttcagctgctccgtgatgcacgaggccctgcacaatcactacacccagaagagcctgagcctgtcccctggcaag

SEQ ID NO: 49 - protein, 451 aa, Artificial Sequence
  Humansed antibody sequence
QVQLVQSGAEVKKPGSSVKVSCKGSGYTFTNYWMHWVRQAPGQGLEWMGATYRGHSDTYYNQKFKGRVTITADTSTSTAYMELSSLRSEDTAVYYCTRGAIYNGYDVLDNWGQGTLVTVSSASTKGPSVFPLAPSSKSTSGGTAALGCLVKDYFPEPVTVSWNSGALTSGVHTFPAVLQSSGLYSLSSVVTVPSSSLGTQTYICNVNHKPSNTKVDKKVEPKSCDKTHTCPPCPAPELLGGPSVFLFPPKPKDTLMISRTPEVTCVVVDVSHEDPEVKFNWYVDGVEVHNAKTKPREEQYNSTYRVVSVLTVLHQDWLNGKEYKCKVSNKALPAPIEKTISKAKGQPREPQVYTLPPSRDELTKNQVSLTCLVKGFYPSDIAVEWESNGQPENNYKTTPPVLDSDGSFFLYSKLTVDKSRWQQGNVFSCSVMHEALHNHYTQKSLSLSPGK

SEQ ID NO: 50 - DNA, 1353 bp, Artificial Sequence
  Humansed antibody sequence
caggtgcagctggtccagagcggcgccgaagtgaagaagcccggcagctccgtgaaagtgagctgcaagggcagcggctacaccttcaccaactactggatgcactgggtgaggcaggcccccggacagggcctggagtggatgggcgccacctacaggggccacagcgacacctactacaaccagaagttcaagggccgggtgaccatcaccgccgacacgagcaccagcaccgcctacatggaactgagcagcctcaggagcgaggacaccgctgtgtattactgcaccaggggcgccatctacaacggctacgacgtgctggacaactggggccagggcacactagtgaccgtgtccagcgccagcaccaagggccccagcgtgttccccctggcccccagcagcaagagcaccagcggcggcacagccgccctgggctgcctggtgaaggactacttccccgaaccggtgaccgtgtcctggaacagcggagccctgaccagcggcgtgcacaccttccccgccgtgctgcagagcagcggcctgtacagcctgagcagcgtggtgaccgtgcccagcagcagcctgggcacccagacctacatctgtaacgtgaaccacaagcccagcaacaccaaggtggacaagaaggtggagcccaagagctgtgacaagacccacacctgccccccctgccctgcccccgagctgctgggaggccccagcgtgttcctgttcccccccaagcctaaggacaccctgatgatcagcagaacccccgaggtgacctgtgtggtggtggatgtgagccacgaggaccctgaggtgaagttcaactggtacgtggacggcgtggaggtgcacaatgccaagaccaagcccagggaggagcagtacaacagcacctaccgggtggtgtccgtgctgaccgtgctgcaccaggattggctgaacggcaaggagtacaagtgtaaggtgtccaacaaggccctgcctgcccctatcgagaaaaccatcagcaaggccaagggccagcccagagagccccaggtgtacaccctgccccctagcagagatgagctgaccaagaaccaggtgtccctgacctgcctggtgaagggcttctaccccagcgacatcgccgtggagtgggagagcaacggccagcccgagaacaactacaagaccaccccccctgtgctggacagcgatggcagcttcttcctgtacagcaagctgaccgtggacaagagcagatggcagcagggcaacgtgttcagctgctccgtgatgcacgaggccctgcacaatcactacacccagaagagcctgagcctgtcccctggcaag

SEQ ID NO: 51 - protein, 451 aa, Artificial Sequence
  Humansed antibody sequence
QVQLVQSGAEVKKPGSSVKVSCKGSGYTFTNYWMHWVRQAPGQGLEWIGATYRGHSDTYYNQKFKGRATLTADTSTSTAYMELSSLRSEDTAVYYCTRGAIYNGYDVLDNWGQGTLVTVSSASTKGPSVFPLAPSSKSTSGGTAALGCLVKDYFPEPVTVSWNSGALTSGVHTFPAVLQSSGLYSLSSVVTVPSSSLGTQTYICNVNHKPSNTKVDKKVEPKSCDKTHTCPPCPAPELLGGPSVFLFPPKPKDTLMISRTPEVTCVVVDVSHEDPEVKFNWYVDGVEVHNAKTKPREEQYNSTYRVVSVLTVLHQDWLNGKEYKCKVSNKALPAPIEKTISKAKGQPREPQVYTLPPSRDELTKNQVSLTCLVKGFYPSDIAVEWESNGQPENNYKTTPPVLDSDGSFFLYSKLTVDKSRWQQGNVFSCSVMHEALHNHYTQKSLSLSPGK

SEQ ID NO: 52 - DNA, 1353 bp, Artificial Sequence
  Humansed antibody sequence
caggtgcagctggtccagagcggcgccgaagtgaagaagcccggcagctccgtgaaagtgagctgcaagggcagcggctacaccttcaccaactactggatgcactgggtgaggcaggcccccggacagggcctggagtggatcggcgccacctacaggggccacagcgacacctactacaaccagaagttcaagggccgggcgaccctcaccgccgacacgagcaccagcaccgcctacatggaactgagcagcctcaggagcgaggacaccgctgtgtattactgcaccaggggcgccatctacaacggctacgacgtgctggacaactggggccagggcacactagtgaccgtgtccagcgccagcaccaagggccccagcgtgttccccctggcccccagcagcaagagcaccagcggcggcacagccgccctgggctgcctggtgaaggactacttccccgaaccggtgaccgtgtcctggaacagcggagccctgaccagcggcgtgcacaccttccccgccgtgctgcagagcagcggcctgtacagcctgagcagcgtggtgaccgtgcccagcagcagcctgggcacccagacctacatctgtaacgtgaaccacaagcccagcaacaccaaggtggacaagaaggtggagcccaagagctgtgacaagacccacacctgccccccctgccctgcccccgagctgctgggaggccccagcgtgttcctgttcccccccaagcctaaggacaccctgatgatcagcagaacccccgaggtgacctgtgtggtggtggatgtgagccacgaggaccctgaggtgaagttcaactggtacgtggacggcgtggaggtgcacaatgccaagaccaagcccagggaggagcagtacaacagcacctaccgggtggtgtccgtgctgaccgtgctgcaccaggattggctgaacggcaaggagtacaagtgtaaggtgtccaacaaggccctgcctgcccctatcgagaaaaccatcagcaaggccaagggccagcccagagagccccaggtgtacaccctgccccctagcagagatgagctgaccaagaaccaggtgtccctgacctgcctggtgaagggcttctaccccagcgacatcgccgtggagtgggagagcaacggccagcccgagaacaactacaagaccaccccccctgtgctggacagcgatggcagcttcttcctgtacagcaagctgaccgtggacaagagcagatggcagcagggcaacgtgttcagctgctccgtgatgcacgaggccctgcacaatcactacacccagaagagcctgagcctgtcccctggcaag

SEQ ID NO: 53 - protein, 451 aa, Artificial Sequence
  Humansed antibody sequence
QVQLVQSGAEVKKPGSSVKVSCKGSGYTFTNYWMHWVRQAPGQGLEWMGATYRGHSDTYYNQKFKGRVTITADTSTSTAYMELSSLRSEDTAVYYCTRGAIYDGYDVLDNWGQGTLVTVSSASTKGPSVFPLAPSSKSTSGGTAALGCLVKDYFPEPVTVSWNSGALTSGVHTFPAVLQSSGLYSLSSVVTVPSSSLGTQTYICNVNHKPSNTKVDKKVEPKSCDKTHTCPPCPAPELLGGPSVFLFPPKPKDTLMISRTPEVTCVVVDVSHEDPEVKFNWYVDGVEVHNAKTKPREEQYNSTYRVVSVLTVLHQDWLNGKEYKCKVSNKALPAPIEKTISKAKGQPREPQVYTLPPSRDELTKNQVSLTCLVKGFYPSDIAVEWESNGQPENNYKTTPPVLDSDGSFFLYSKLTVDKSRWQQGNVFSCSVMHEALHNHYTQKSLSLSPGK

SEQ ID NO: 54 - DNA, 1353 bp, Artificial Sequence
  Humansed antibody sequence
caggtgcagctggtccagagcggcgccgaagtgaagaagcccggcagctccgtgaaagtgagctgcaagggcagcggctacaccttcaccaactactggatgcactgggtgaggcaggcccccggacagggcctggagtggatgggcgccacctacaggggccacagcgacacctactacaaccagaagttcaagggccgggtgaccatcaccgccgacacgagcaccagcaccgcctacatggaactgagcagcctcaggagcgaggacaccgctgtgtattactgcaccaggggcgccatctacgacggctacgacgtgctggacaactggggccagggcacactagtgaccgtgtccagcgccagcaccaagggccccagcgtgttccccctggcccccagcagcaagagcaccagcggcggcacagccgccctgggctgcctggtgaaggactacttccccgaaccggtgaccgtgtcctggaacagcggagccctgaccagcggcgtgcacaccttccccgccgtgctgcagagcagcggcctgtacagcctgagcagcgtggtgaccgtgcccagcagcagcctgggcacccagacctacatctgtaacgtgaaccacaagcccagcaacaccaaggtggacaagaaggtggagcccaagagctgtgacaagacccacacctgccccccctgccctgcccccgagctgctgggaggccccagcgtgttcctgttcccccccaagcctaaggacaccctgatgatcagcagaacccccgaggtgacctgtgtggtggtggatgtgagccacgaggaccctgaggtgaagttcaactggtacgtggacggcgtggaggtgcacaatgccaagaccaagcccagggaggagcagtacaacagcacctaccgggtggtgtccgtgctgaccgtgctgcaccaggattggctgaacggcaaggagtacaagtgtaaggtgtccaacaaggccctgcctgcccctatcgagaaaaccatcagcaaggccaagggccagcccagagagccccaggtgtacaccctgccccctagcagagatgagctgaccaagaaccaggtgtccctgacctgcctggtgaagggcttctaccccagcgacatcgccgtggagtgggagagcaacggccagcccgagaacaactacaagaccaccccccctgtgctggacagcgatggcagcttcttcctgtacagcaagctgaccgtggacaagagcagatggcagcagggcaacgtgttcagctgctccgtgatgcacgaggccctgcacaatcactacacccagaagagcctgagcctgtcccctggcaag

SEQ ID NO: 55 - protein, 451 aa, Artificial Sequence
  Humansed antibody sequence
QVQLVQSGAEVKKPGSSVKVSCKASGGTFSNYWMHWVRQAPGQGLEWMGATYRGHSDTYYNQKFKGRVTITADKSTSTAYMELSSLRSEDTAVYYCARGAIYDGYDVLDNWGQGTLVTVSSASTKGPSVFPLAPSSKSTSGGTAALGCLVKDYFPEPVTVSWNSGALTSGVHTFPAVLQSSGLYSLSSVVTVPSSSLGTQTYICNVNHKPSNTKVDKKVEPKSCDKTHTCPPCPAPELLGGPSVFLFPPKPKDTLMISRTPEVTCVVVDVSHEDPEVKFNWYVDGVEVHNAKTKPREEQYNSTYRVVSVLTVLHQDWLNGKEYKCKVSNKALPAPIEKTISKAKGQPREPQVYTLPPSRDELTKNQVSLTCLVKGFYPSDIAVEWESNGQPENNYKTTPPVLDSDGSFFLYSKLTVDKSRWQQGNVFSCSVMHEALHNHYTQKSLSLSPGK

SEQ ID NO: 56 - DNA, 1353 bp, Artificial Sequence
  Humansed antibody sequence
caggtgcagctggtccagagcggcgccgaagtgaagaagcccggcagctccgtgaaagtgagctgcaaggccagcggcggcaccttcagcaactactggatgcactgggtgaggcaggcccccggacagggcctggagtggatgggcgccacctacaggggccacagcgacacctactacaaccagaagttcaagggccgggtgaccatcaccgccgacaagagcaccagcaccgcctacatggaactgagcagcctcaggagcgaggacaccgctgtgtattactgcgccaggggcgccatctacgacggctacgacgtgctggacaactggggccagggcacactagtgaccgtgtccagcgccagcaccaagggccccagcgtgttccccctggcccccagcagcaagagcaccagcggcggcacagccgccctgggctgcctggtgaaggactacttccccgaaccggtgaccgtgtcctggaacagcggagccctgaccagcggcgtgcacaccttccccgccgtgctgcagagcagcggcctgtacagcctgagcagcgtggtgaccgtgcccagcagcagcctgggcacccagacctacatctgtaacgtgaaccacaagcccagcaacaccaaggtggacaagaaggtggagcccaagagctgtgacaagacccacacctgccccccctgccctgcccccgagctgctgggaggccccagcgtgttcctgttcccccccaagcctaaggacaccctgatgatcagcagaacccccgaggtgacctgtgtggtggtggatgtgagccacgaggaccctgaggtgaagttcaactggtacgtggacggcgtggaggtgcacaatgccaagaccaagcccagggaggagcagtacaacagcacctaccgggtggtgtccgtgctgaccgtgctgcaccaggattggctgaacggcaaggagtacaagtgtaaggtgtccaacaaggccctgcctgcccctatcgagaaaaccatcagcaaggccaagggccagcccagagagccccaggtgtacaccctgccccctagcagagatgagctgaccaagaaccaggtgtccctgacctgcctggtgaagggcttctaccccagcgacatcgccgtggagtgggagagcaacggccagcccgagaacaactacaagaccaccccccctgtgctggacagcgatggcagcttcttcctgtacagcaagctgaccgtggacaagagcagatggcagcagggcaacgtgttcagctgctccgtgatgcacgaggccctgcacaatcactacacccagaagagcctgagcctgtcccctggcaag

SEQ ID NO: 57 - protein, 451 aa, Artificial Sequence
  Humansed antibody sequence
QVQLVQSGAEVKKPGSSVKVSCKASGYTFTNYWMHWVRQAPGQGLEWMGATYRGHSDTYYNQKFKGRVTITADKSTSTAYMELSSLRSEDTAVYYCARGAIYDGYDVLDNWGQGTLVTVSSASTKGPSVFPLAPSSKSTSGGTAALGCLVKDYFPEPVTVSWNSGALTSGVHTFPAVLQSSGLYSLSSVVTVPSSSLGTQTYICNVNHKPSNTKVDKKVEPKSCDKTHTCPPCPAPELLGGPSVFLFPPKPKDTLMISRTPEVTCVVVDVSHEDPEVKFNWYVDGVEVHNAKTKPREEQYNSTYRVVSVLTVLHQDWLNGKEYKCKVSNKALPAPIEKTISKAKGQPREPQVYTLPPSRDELTKNQVSLTCLVKGFYPSDIAVEWESNGQPENNYKTTPPVLDSDGSFFLYSKLTVDKSRWQQGNVFSCSVMHEALHNHYTQKSLSLSPGK

SEQ ID NO: 58 - DNA, 1353 bp, Artificial Sequence
  Humansed antibody sequence
caggtgcagctggtccagagcggcgccgaagtgaagaagcccggcagctccgtgaaagtgagctgcaaggccagcggctacaccttcaccaactactggatgcactgggtgaggcaggcccccggacagggcctggagtggatgggcgccacctacaggggccacagcgacacctactacaaccagaagttcaagggccgggtgaccatcaccgccgacaagagcaccagcaccgcctacatggaactgagcagcctcaggagcgaggacaccgctgtgtattactgcgccaggggcgccatctacgacggctacgacgtgctggacaactggggccagggcacactagtgaccgtgtccagcgccagcaccaagggccccagcgtgttccccctggcccccagcagcaagagcaccagcggcggcacagccgccctgggctgcctggtgaaggactacttccccgaaccggtgaccgtgtcctggaacagcggagccctgaccagcggcgtgcacaccttccccgccgtgctgcagagcagcggcctgtacagcctgagcagcgtggtgaccgtgcccagcagcagcctgggcacccagacctacatctgtaacgtgaaccacaagcccagcaacaccaaggtggacaagaaggtggagcccaagagctgtgacaagacccacacctgccccccctgccctgcccccgagctgctgggaggccccagcgtgttcctgttcccccccaagcctaaggacaccctgatgatcagcagaacccccgaggtgacctgtgtggtggtggatgtgagccacgaggaccctgaggtgaagttcaactggtacgtggacggcgtggaggtgcacaatgccaagaccaagcccagggaggagcagtacaacagcacctaccgggtggtgtccgtgctgaccgtgctgcaccaggattggctgaacggcaaggagtacaagtgtaaggtgtccaacaaggccctgcctgcccctatcgagaaaaccatcagcaaggccaagggccagcccagagagccccaggtgtacaccctgccccctagcagagatgagctgaccaagaaccaggtgtccctgacctgcctggtgaagggcttctaccccagcgacatcgccgtggagtgggagagcaacggccagcccgagaacaactacaagaccaccccccctgtgctggacagcgatggcagcttcttcctgtacagcaagctgaccgtggacaagagcagatggcagcagggcaacgtgttcagctgctccgtgatgcacgaggccctgcacaatcactacacccagaagagcctgagcctgtcccctggcaag

SEQ ID NO: 59 - protein, 451 aa, Artificial Sequence
  Humansed antibody sequence
QVQLVQSGAEVKKPGSSVKVSCKASGYTFTNYWMHWVRQAPGQGLEWMGATYRGHSDTYYNQKFKGRVTITADKSTSTAYMELSSLRSEDTAVYYCTRGAIYDGYDVLDNWGQGTLVTVSSASTKGPSVFPLAPSSKSTSGGTAALGCLVKDYFPEPVTVSWNSGALTSGVHTFPAVLQSSGLYSLSSVVTVPSSSLGTQTYICNVNHKPSNTKVDKKVEPKSCDKTHTCPPCPAPELLGGPSVFLFPPKPKDTLMISRTPEVTCVVVDVSHEDPEVKFNWYVDGVEVHNAKTKPREEQYNSTYRVVSVLTVLHQDWLNGKEYKCKVSNKALPAPIEKTISKAKGQPREPQVYTLPPSRDELTKNQVSLTCLVKGFYPSDIAVEWESNGQPENNYKTTPPVLDSDGSFFLYSKLTVDKSRWQQGNVFSCSVMHEALHNHYTQKSLSLSPGK

SEQ ID NO: 60 - DNA, 1353 bp, Artificial Sequence
  Humansed antibody sequence
caggtgcagctggtccagagcggcgccgaagtgaagaagcccggcagctccgtgaaagtgagctgcaaggccagcggctacaccttcaccaactactggatgcactgggtgaggcaggcccccggacagggcctggagtggatgggcgccacctacaggggccacagcgacacctactacaaccagaagttcaagggccgggtgaccatcaccgccgacaagagcaccagcaccgcctacatggaactgagcagcctcaggagcgaggacaccgctgtgtattactgcaccaggggcgccatctacgacggctacgacgtgctggacaactggggccagggcacactagtgaccgtgtccagcgccagcaccaagggccccagcgtgttccccctggcccccagcagcaagagcaccagcggcggcacagccgccctgggctgcctggtgaaggactacttccccgaaccggtgaccgtgtcctggaacagcggagccctgaccagcggcgtgcacaccttccccgccgtgctgcagagcagcggcctgtacagcctgagcagcgtggtgaccgtgcccagcagcagcctgggcacccagacctacatctgtaacgtgaaccacaagcccagcaacaccaaggtggacaagaaggtggagcccaagagctgtgacaagacccacacctgccccccctgccctgcccccgagctgctgggaggccccagcgtgttcctgttcccccccaagcctaaggacaccctgatgatcagcagaacccccgaggtgacctgtgtggtggtggatgtgagccacgaggaccctgaggtgaagttcaactggtacgtggacggcgtggaggtgcacaatgccaagaccaagcccagggaggagcagtacaacagcacctaccgggtggtgtccgtgctgaccgtgctgcaccaggattggctgaacggcaaggagtacaagtgtaaggtgtccaacaaggccctgcctgcccctatcgagaaaaccatcagcaaggccaagggccagcccagagagccccaggtgtacaccctgccccctagcagagatgagctgaccaagaaccaggtgtccctgacctgcctggtgaagggcttctaccccagcgacatcgccgtggagtgggagagcaacggccagcccgagaacaactacaagaccaccccccctgtgctggacagcgatggcagcttcttcctgtacagcaagctgaccgtggacaagagcagatggcagcagggcaacgtgttcagctgctccgtgatgcacgaggccctgcacaatcactacacccagaagagcctgagcctgtcccctggcaag

SEQ ID NO: 61 - protein, 451 aa, Artificial Sequence
  Humansed antibody sequence
QVQLVQSGAEVKKPGSSVKVSCKGSGYTFTNYWMHWVRQAPGQGLEWIGATYRGHSDTYYNQKFKGRATLTADTSTSTAYMELSSLRSEDTAVYYCTRGAIYDGYDVLDNWGQGTLVTVSSASTKGPSVFPLAPSSKSTSGGTAALGCLVKDYFPEPVTVSWNSGALTSGVHTFPAVLQSSGLYSLSSVVTVPSSSLGTQTYICNVNHKPSNTKVDKKVEPKSCDKTHTCPPCPAPELLGGPSVFLFPPKPKDTLMISRTPEVTCVVVDVSHEDPEVKFNWYVDGVEVHNAKTKPREEQYNSTYRVVSVLTVLHQDWLNGKEYKCKVSNKALPAPIEKTISKAKGQPREPQVYTLPPSRDELTKNQVSLTCLVKGFYPSDIAVEWESNGQPENNYKTTPPVLDSDGSFFLYSKLTVDKSRWQQGNVFSCSVMHEALHNHYTQKSLSLSPGK

SEQ ID NO: 62 - DNA, 1353 bp, Artificial Sequence
  Humansed antibody sequence
caggtgcagctggtccagagcggcgccgaagtgaagaagcccggcagctccgtgaaagtgagctgcaagggcagcggctacaccttcaccaactactggatgcactgggtgaggcaggcccccggacagggcctggagtggatcggcgccacctacaggggccacagcgacacctactacaaccagaagttcaagggccgggcgaccctcaccgccgacacgagcaccagcaccgcctacatggaactgagcagcctcaggagcgaggacaccgctgtgtattactgcaccaggggcgccatctacgacggctacgacgtgctggacaactggggccagggcacactagtgaccgtgtccagcgccagcaccaagggccccagcgtgttccccctggcccccagcagcaagagcaccagcggcggcacagccgccctgggctgcctggtgaaggactacttccccgaaccggtgaccgtgtcctggaacagcggagccctgaccagcggcgtgcacaccttccccgccgtgctgcagagcagcggcctgtacagcctgagcagcgtggtgaccgtgcccagcagcagcctgggcacccagacctacatctgtaacgtgaaccacaagcccagcaacaccaaggtggacaagaaggtggagcccaagagctgtgacaagacccacacctgccccccctgccctgcccccgagctgctgggaggccccagcgtgttcctgttcccccccaagcctaaggacaccctgatgatcagcagaacccccgaggtgacctgtgtggtggtggatgtgagccacgaggaccctgaggtgaagttcaactggtacgtggacggcgtggaggtgcacaatgccaagaccaagcccagggaggagcagtacaacagcacctaccgggtggtgtccgtgctgaccgtgctgcaccaggattggctgaacggcaaggagtacaagtgtaaggtgtccaacaaggccctgcctgcccctatcgagaaaaccatcagcaaggccaagggccagcccagagagccccaggtgtacaccctgccccctagcagagatgagctgaccaagaaccaggtgtccctgacctgcctggtgaagggcttctaccccagcgacatcgccgtggagtgggagagcaacggccagcccgagaacaactacaagaccaccccccctgtgctggacagcgatggcagcttcttcctgtacagcaagctgaccgtggacaagagcagatggcagcagggcaacgtgttcagctgctccgtgatgcacgaggccctgcacaatcactacacccagaagagcctgagcctgtcccctggcaag

SEQ ID NO: 63 - protein, 214 aa, Artificial Sequence
  Humansed antibody sequence
DIQMTQSPSSLSASVGDRVTITCSASQDISNYLNWYQQKPGKAPKLLIYYTSNLHSGVPSRFSGSGSGTDFTLTISSLQPEDFATYYCQQYRKLPWTFGQGTKLEIKRTVAAPSVFIFPPSDEQLKSGTASVVCLLNNFYPREAKVQWKVDNALQSGNSQESVTEQDSKDSTYSLSSTLTLSKADYEKHKVYACEVTHQGLSSPVTKSFNRGEC

SEQ ID NO: 64 - DNA, 642 bp, Artificial Sequence
  Humansed antibody sequence
gacatccagatgacccagagccctagctcactgagcgccagcgtgggcgacagggtgaccattacctgctccgccagccaggacatcagcaactacctgaactggtaccagcagaagcccggcaaggcccccaagctgctgatctactacacctccaacctgcactccggcgtgcccagcaggttcagcggaagcggcagcggcaccgatttcaccctgaccatctccagcctgcagcccgaggacttcgccacctactactgccagcagtacaggaagctcccctggactttcggccagggcaccaaactggagatcaagcgtacggtggccgcccccagcgtgttcatcttcccccccagcgatgagcagctgaagagcggcaccgccagcgtggtgtgtctgctgaacaacttctacccccgggaggccaaggtgcagtggaaggtggacaatgccctgcagagcggcaacagccaggagagcgtgaccgagcaggacagcaaggactccacctacagcctgagcagcaccctgaccctgagcaaggccgactacgagaagcacaaggtgtacgcctgtgaggtgacccaccagggcctgtccagccccgtgaccaagagcttcaaccggggcgagtgc

SEQ ID NO: 65 - protein, 214 aa, Artificial Sequence
  Humansed antibody sequence
DIQMTQSPSSLSASVGDRVTITCSASQDISNYLNWYQQKPGKAPKLLIYYTSNLHSGVPSRFSGSGSGTDYTLTISSLQPEDFATYYCQQYRKLPWTFGQGTKLEIKRTVAAPSVFIFPPSDEQLKSGTASVVCLLNNFYPREAKVQWKVDNALQSGNSQESVTEQDSKDSTYSLSSTLTLSKADYEKHKVYACEVTHQGLSSPVTKSFNRGEC

SEQ ID NO: 66 - DNA, 642 bp, Artificial Sequence
  Humansed antibody sequence
gacatccagatgacccagagccctagctcactgagcgccagcgtgggcgacagggtgaccattacctgctccgccagccaggacatcagcaactacctgaactggtaccagcagaagcccggcaaggcccccaagctgctgatctactacacctccaacctgcactccggcgtgcccagcaggttcagcggaagcggcagcggcaccgattacaccctgaccatctccagcctgcagcccgaggacttcgccacctactactgccagcagtacaggaagctcccctggactttcggccagggcaccaaactggagatcaagcgtacggtggccgcccccagcgtgttcatcttcccccccagcgatgagcagctgaagagcggcaccgccagcgtggtgtgtctgctgaacaacttctacccccgggaggccaaggtgcagtggaaggtggacaatgccctgcagagcggcaacagccaggagagcgtgaccgagcaggacagcaaggactccacctacagcctgagcagcaccctgaccctgagcaaggccgactacgagaagcacaaggtgtacgcctgtgaggtgacccaccagggcctgtccagccccgtgaccaagagcttcaaccggggcgagtgc

SEQ ID NO: 67 - protein, 214 aa, Artificial Sequence
  Humansed antibody sequence
DIQLTQSPSSLSASVGDRVTITCSASQDISNYLNWYQQKPGKAPELVIYYTSNLHSGVPSRFSGSGSGTDYTLTISSLQPEDFATYYCQQYRKLPWTFGQGTKLEIKRTVAAPSVFIFPPSDEQLKSGTASVVCLLNNFYPREAKVQWKVDNALQSGNSQESVTEQDSKDSTYSLSSTLTLSKADYEKHKVYACEVTHQGLSSPVTKSFNRGEC

SEQ ID NO: 68 - DNA, 642 bp, Artificial Sequence
  Humansed antibody sequence
gacatccagctgacccagagccctagctcactgagcgccagcgtgggcgacagggtgaccattacctgctccgccagccaggacatcagcaactacctgaactggtaccagcagaagcccggcaaggcccccgagctggtgatctactacacctccaacctgcactccggcgtgcccagcaggttcagcggaagcggcagcggcaccgattacaccctgaccatctccagcctgcagcccgaggacttcgccacctactactgccagcagtacaggaagctcccctggactttcggccagggcaccaaactggagatcaagcgtacggtggccgcccccagcgtgttcatcttcccccccagcgatgagcagctgaagagcggcaccgccagcgtggtgtgtctgctgaacaacttctacccccgggaggccaaggtgcagtggaaggtggacaatgccctgcagagcggcaacagccaggagagcgtgaccgagcaggacagcaaggactccacctacagcctgagcagcaccctgaccctgagcaaggccgactacgagaagcacaaggtgtacgcctgtgaggtgacccaccagggcctgtccagccccgtgaccaagagcttcaaccggggcgagtgc

SEQ ID NO: 69 - protein, 115 aa, mus musculus
EVQLQQSGPELVKPGASVKISCKASGYTFTDYYMKWVKQSHGKSLEWIGEIYPNNGGITYNQKFKGKATLTVDKSSSTAYMELRSLTSEDSAVYYCANGYEFVYWGQGTLVTVSA

SEQ ID NO: 70 - DNA, 345 bp, mus musculus
gaggtccagttgcaacaatctggacctgagctggtgaagcctggggcttcagtgaagatatcctgtaaggcttctggatacacattcactgactactacatgaagtgggtgaagcagagccatggaaagagccttgagtggattggagagatttatcctaataatggtggtattacctacaaccagaagttcaagggcaaggccacattgactgtagacaagtcctccagcacagcctacatggagctccgcagcctgacatctgaggactctgcagtctattactgtgcaaatggttacgagtttgtttactggggccaagggactctggtcactgtctctgca

SEQ ID NO: 71 - protein, 108 aa, mus musculus
DIQMTQTASSLSASLGDRVTISCSASQGISNYLNWYQQKPDGTVKLLIYYTSSLHSGVPSRFSGSGSGTDYSLTISNLEPEDIATYYCQQYSKLPWTFGGGTKLEIKR

SEQ ID NO: 72 - DNA, 324 bp, mus musculus
gatatccagatgacacagactgcatcctccctgtctgcctctctgggagacagagtcaccatcagttgcagtgcaagtcagggcattagcaattatttaaactggtatcagcagaaaccagatggaactgttaaactcctgatctattacacatcaagtttacactcaggagtcccatcaaggttcagtggcagtgggtctgggacagattattctctcaccatcagcaacctggaacctgaagatattgccacttactattgtcagcagtatagtaagcttccgtggacgttcggtggaggcaccaagctggaaatcaaacgg

SEQ ID NO: 73 - protein, 445 aa, Artificial Sequence
  Chimeric antibody sequence
EVQLQQSGPELVKPGASVKISCKASGYTFTDYYMKWVKQSHGKSLEWIGEIYPNNGGITYNQKFKGKATLTVDKSSSTAYMELRSLTSEDSAVYYCANGYEFVYWGQGTLVTVSAAKTTAPSVFPLAPSSKSTSGGTAALGCLVKDYFPEPVTVSWNSGALTSGVHTFPAVLQSSGLYSLSSVVTVPSSSLGTQTYICNVNHKPSNTKVDKKVEPKSCDKTHTCPPCPAPELLGGPSVFLFPPKPKDTLMISRTPEVTCVVVDVSHEDPEVKFNWYVDGVEVHNAKTKPREEQYNSTYRVVSVLTVLHQDWLNGKEYKCKVSNKALPAPIEKTISKAKGQPREPQVYTLPPSRDELTKNQVSLTCLVKGFYPSDIAVEWESNGQPENNYKTTPPVLDSDGSFFLYSKLTVDKSRWQQGNVFSCSVMHEALHNHYTQKSLSLSPGK

SEQ ID NO: 74 - DNA, 1335 bp, Artificial Sequence
  Chimeric antibody sequence
gaggtccagttgcaacaatctggacctgagctggtgaagcctggggcttcagtgaagatatcctgtaaggcttctggatacacattcactgactactacatgaagtgggtgaagcagagccatggaaagagccttgagtggattggagagatttatcctaataatggtggtattacctacaaccagaagttcaagggcaaggccacattgactgtagacaagtcctccagcacagcctacatggagctccgcagcctgacatctgaggactctgcagtctattactgtgcaaatggttacgagtttgtttactggggccaagggactctggtcactgtctctgcagccaaaacaacagcccccagcgtgttccccctggcccccagcagcaagagcaccagcggcggcacagccgccctgggctgcctggtgaaggactacttccccgaaccggtgaccgtgtcctggaacagcggagccctgaccagcggcgtgcacaccttccccgccgtgctgcagagcagcggcctgtacagcctgagcagcgtggtgaccgtgcccagcagcagcctgggcacccagacctacatctgtaacgtgaaccacaagcccagcaacaccaaggtggacaagaaggtggagcccaagagctgtgacaagacccacacctgccccccctgccctgcccccgagctgctgggaggccccagcgtgttcctgttcccccccaagcctaaggacaccctgatgatcagcagaacccccgaggtgacctgtgtggtggtggatgtgagccacgaggaccctgaggtgaagttcaactggtacgtggacggcgtggaggtgcacaatgccaagaccaagcccagggaggagcagtacaacagcacctaccgggtggtgtccgtgctgaccgtgctgcaccaggattggctgaacggcaaggagtacaagtgtaaggtgtccaacaaggccctgcctgcccctatcgagaaaaccatcagcaaggccaagggccagcccagagagccccaggtgtacaccctgccccctagcagagatgagctgaccaagaaccaggtgtccctgacctgcctggtgaagggcttctaccccagcgacatcgccgtggagtgggagagcaacggccagcccgagaacaactacaagaccaccccccctgtgctggacagcgatggcagcttcttcctgtacagcaagctgaccgtggacaagagcagatggcagcagggcaacgtgttcagctgctccgtgatgcacgaggccctgcacaatcactacacccagaagagcctgagcctgtcccctggcaag

SEQ ID NO: 75 - protein, 214 aa, Artificial Sequence
  Chimeric antibody sequence
DIQMTQTASSLSASLGDRVTISCSASQGISNYLNWYQQKPDGTVKLLIYYTSSLHSGVPSRFSGSGSGTDYSLTISNLEPEDIATYYCQQYSKLPWTFGGGTKLELKRTVAAPSVFIFPPSDEQLKSGTASVVCLLNNFYPREAKVQWKVDNALQSGNSQESVTEQDSKDSTYSLSSTLTLSKADYEKHKVYACEVTHQGLSSPVTKSFNRGEC

SEQ ID NO: 76 - DNA, 642 bp, Artificial Sequence
  Chimeric antibody sequence
gatatccagatgacacagactgcatcctccctgtctgcctctctgggagacagagtcaccatcagttgcagtgcaagtcagggcattagcaattatttaaactggtatcagcagaaaccagatggaactgttaaactcctgatctattacacatcaagtttacactcaggagtcccatcaaggttcagtggcagtgggtctgggacagattattctctcaccatcagcaacctggaacctgaagatattgccacttactattgtcagcagtatagtaagcttccgtggacgttcggtggaggcaccaagctggagctgaaacgtacggtggccgcccccagcgtgttcatcttcccccccagcgatgagcagctgaagagcggcaccgccagcgtggtgtgtctgctgaacaacttctacccccgggaggccaaggtgcagtggaaggtggacaatgccctgcagagcggcaacagccaggagagcgtgaccgagcaggacagcaaggactccacctacagcctgagcagcaccctgaccctgagcaaggccgactacgagaagcacaaggtgtacgcctgtgaggtgacccaccagggcctgtccagccccgtgaccaagagcttcaaccggggcgagtgc

SEQ ID NO: 77 - protein, 115 aa, Artificial Sequence
  Humansed antibody sequence
QVQLVQSGAEVKKPGSSVKVSCKASGGTFSDYYMKWVRQAPGQGLEWMGEIYPNNGGITYNQKFKGRVTITADKSTSTAYMELSSLRSEDTAVYYCARGYEFVYWGQGTLVTVSS

SEQ ID NO: 78 - DNA, 345 bp, Artificial Sequence
  Humansed antibody sequence
caggtgcagctggtgcagagcggcgccgaagtgaagaagcccggctccagcgtgaaggtgagctgcaaggctagcggcggcaccttcagcgactactacatgaagtgggtgaggcaggcccccggccagggactggagtggatgggcgagatctaccccaacaacgggggcatcacctacaaccagaagttcaagggcagggtgaccatcaccgccgacaaaagcaccagcaccgcctacatggaactgagcagcctgaggagcgaggacaccgccgtgtactactgcgccaggggctacgagttcgtgtattggggccagggcacactagtgaccgtgtccagc

SEQ ID NO: 79 - protein, 115 aa, Artificial Sequence
  Humansed antibody sequence
QVQLVQSGAEVKKPGSSVKVSCKASGYTFTDYYMKWVRQAPGQGLEWMGEIYPNNGGITYNQKFKGRVTITADKSTSTAYMELSSLRSEDTAVYYCARGYEFVYWGQGTLVTVSS

SEQ ID NO: 80 - DNA, 345 bp, Artificial Sequence
  Humansed antibody sequence
caggtgcagctggtgcagagcggcgccgaagtgaagaagcccggctccagcgtgaaggtgagctgcaaggctagcggctacaccttcaccgactactacatgaagtgggtgaggcaggcccccggccagggactggagtggatgggcgagatctaccccaacaacgggggcatcacctacaaccagaagttcaagggcagggtgaccatcaccgccgacaaaagcaccagcaccgcctacatggaactgagcagcctgaggagcgaggacaccgccgtgtactactgcgccaggggctacgagttcgtgtattggggccagggcacactagtgaccgtgtccagc

SEQ ID NO: 81 - protein, 115 aa, Artificial Sequence
  Humansed antibody sequence
QVQLVQSGAEVKKPGSSVKVSCKASGYTFTDYYMKWVRQAPGQGLEWMGEIYPNNGGITYNQKFKGRVTITADKSTSTAYMELSSLRSEDTAVYYCANGYEFVYWGQGTLVTVSS

SEQ ID NO: 82 - DNA, 345 bp, Artificial Sequence
  Humansed antibody sequence
caggtgcagctggtgcagagcggcgccgaagtgaagaagcccggctccagcgtgaaggtgagctgcaaggctagcggctacaccttcaccgactactacatgaagtgggtgaggcaggcccccggccagggactggagtggatgggcgagatctaccccaacaacgggggcatcacctacaaccagaagttcaagggcagggtgaccatcaccgccgacaaaagcaccagcaccgcctacatggaactgagcagcctgaggagcgaggacaccgccgtgtactactgcgccaacggctacgagttcgtgtattggggccagggcacactagtgaccgtgtccagc

SEQ ID NO: 83 - protein, 115 aa, Artificial Sequence
  Humansed antibody sequence
QVQLVQSGAEVKKPGSSVKVSCKASGYTFTDYYMKWVRQAPGQGLEWIGEIYPNNGGITYNQKFKGRATLTVDKSTSTAYMELSSLRSEDTAVYYCANGYEFVYWGQGTLVTVSS

SEQ ID NO: 84 - DNA, 345 bp, Artificial Sequence
  Humansed antibody sequence
caggtgcagctggtgcagagcggcgccgaagtgaagaagcccggctccagcgtgaaggtgagctgcaaggctagcggctacaccttcaccgactactacatgaagtgggtgaggcaggcccccggccagggactggagtggataggcgagatctaccccaacaacgggggcatcacctacaaccagaagttcaagggcagggcgaccctcaccgtcgacaaaagcaccagcaccgcctacatggaactgagcagcctgaggagcgaggacaccgccgtgtactactgcgccaacggctacgagttcgtgtattggggccagggcacactagtgaccgtgtccagc

SEQ ID NO: 85 - protein, 115 aa, Artificial Sequence
  Humansed antibody sequence
QVQLVQSGAEVKKPGSSVKVSCKASGYTFTDYYMKWVRQAPGQGLEWMGEIYPNNGGITYNQKFKGRVTITADKSTSTAYMELSSLRSEDTAVYYCADGYEFVYWGQGTLVTVSS

SEQ ID NO: 86 - DNA, 345 bp, Artificial Sequence
  Humansed antibody sequence
caggtgcagctggtgcagagcggcgccgaagtgaagaagcccggctccagcgtgaaggtgagctgcaaggctagcggctacaccttcaccgactactacatgaagtgggtgaggcaggcccccggccagggactggagtggatgggcgagatctaccccaacaacgggggcatcacctacaaccagaagttcaagggcagggtgaccatcaccgccgacaaaagcaccagcaccgcctacatggaactgagcagcctgaggagcgaggacaccgccgtgtactactgcgccgacggctacgagttcgtgtattggggccagggcacactagtgaccgtgtccagc

SEQ ID NO: 87 - protein, 115 aa, Artificial Sequence
  Humansed antibody sequence
QVQLVQSGAEVKKPGSSVKVSCKASGYTFTDYYMKWVRQAPGQGLEWIGEIYPNNGGITYNQKFKGRATLTVDKSTSTAYMELSSLRSEDTAVYYCANGYEFDYWGQGTLVTVSS

SEQ ID NO: 88 - DNA, 345 bp, Artificial Sequence
  Humansed antibody sequence
caggtgcagctggtgcagagcggcgccgaagtgaagaagcccggctccagcgtgaaggtgagctgcaaggctagcggctacaccttcaccgactactacatgaagtgggtgaggcaggcccccggccagggactggagtggataggcgagatctaccccaacaacgggggcatcacctacaaccagaagttcaagggcagggcgaccctcaccgtcgacaaaagcaccagcaccgcctacatggaactgagcagcctgaggagcgaggacaccgccgtgtactactgcgccaacggctacgagttcgactattggggccagggcacactagtgaccgtgtccagc

SEQ ID NO: 89 - protein, 108 aa, Artificial Sequence
  Humansed antibody sequence
DIQMTQSPSSLSASVGDRVTITCSASQGISNYLNWYQQKPGKAPKLLIYYTSSLHSGVPSRFSGSGSGTDFTLTISSLQPEDFATYYCQQYSKLPWTFGQGTKLEIKR

SEQ ID NO: 90 - DNA, 324 bp, Artificial Sequence
  Humansed antibody sequence
gacatccagatgacccagagcccctcaagcctgagcgccagcgtgggcgacagggtgactatcacctgcagcgcctcccagggcatcagcaactacctgaactggtaccagcagaagcccggcaaggcccctaagctgctgatctactacaccagcagcctgcacagcggcgtgcccagcaggttctccggcagcggcagcggaaccgacttcaccctgaccattagcagcctccagcccgaggacttcgccacctactactgccagcagtacagcaagctgccctggaccttcggccagggcaccaaactggagatcaagcgt

SEQ ID NO: 91 - protein, 108 aa, Artificial Sequence
  Humansed antibody sequence
DIQMTQSPSSLSASVGDRVTITCSASQGISNYLNWYQQKPGKAPKLLIYYTSSLHSGVPSRFSGSGSGTDYTLTISSLQPEDFATYYCQQYSKLPWTFGQGTKLEIKR

SEQ ID NO: 92 - DNA, 324 bp, Artificial Sequence
  Humansed antibody sequence
gacatccagatgacccagagcccctcaagcctgagcgccagcgtgggcgacagggtgactatcacctgcagcgcctcccagggcatcagcaactacctgaactggtaccagcagaagcccggcaaggcccctaagctgctgatctactacaccagcagcctgcacagcggcgtgcccagcaggttctccggcagcggcagcggaaccgactacaccctgaccattagcagcctccagcccgaggacttcgccacctactactgccagcagtacagcaagctgccctggaccttcggccagggcaccaaactggagatcaagcgt

SEQ ID NO: 93 - protein, 5 aa, mus musculus
DYYMK

SEQ ID NO: 94 - protein, 17 aa, mus musculus
EIYPNNGGITYNQKFKG

SEQ ID NO: 95 - protein, 6 aa, mus musculus
GYEFVY

SEQ ID NO: 96 - protein, 11 aa, mus musculus
SASQGISNYLN

SEQ ID NO: 97 - protein, 7 aa, mus musculus
YTSSLHS

SEQ ID NO: 98 - protein, 9 aa, mus musculus
QQYSKLPWT

SEQ ID NO: 99 - protein, 6 aa, Artificial Sequence
  Humansed antibody sequence
GYEFDY

SEQ ID NO: 100 - protein, 445 aa, Artificial Sequence
  Humansed antibody sequence
QVQLVQSGAEVKKPGSSVKVSCKASGGTFSDYYMKWVRQAPGQGLEWMGEIYPNNGGITYNQKFKGRVTITADKSTSTAYMELSSLRSEDTAVYYCARGYEFVYWGQGTLVTVSSASTKGPSVFPLAPSSKSTSGGTAALGCLVKDYFPEPVTVSWNSGALTSGVHTFPAVLQSSGLYSLSSVVTVPSSSLGTQTYICNVNHKPSNTKVDKKVEPKSCDKTHTCPPCPAPELLGGPSVFLFPPKPKDTLMISRTPEVTCVVVDVSHEDPEVKFNWYVDGVEVHNAKTKPREEQYNSTYRVVSVLTVLHQDWLNGKEYKCKVSNKALPAPIEKTISKAKGQPREPQVYTLPPSRDELTKNQVSLTCLVKGFYPSDIAVEWESNGQPENNYKTTPPVLDSDGSFFLYSKLTVDKSRWQQGNVFSCSVMHEALHNHYTQKSLSLSPGK

SEQ ID NO: 101 - DNA, 1335 bp, Artificial Sequence
  Humansed antibody sequence
caggtgcagctggtgcagagcggcgccgaagtgaagaagcccggctccagcgtgaaggtgagctgcaaggctagcggcggcaccttcagcgactactacatgaagtgggtgaggcaggcccccggccagggactggagtggatgggcgagatctaccccaacaacgggggcatcacctacaaccagaagttcaagggcagggtgaccatcaccgccgacaaaagcaccagcaccgcctacatggaactgagcagcctgaggagcgaggacaccgccgtgtactactgcgccaggggctacgagttcgtgtattggggccagggcacactagtgaccgtgtccagcgccagcaccaagggccccagcgtgttccccctggcccccagcagcaagagcaccagcggcggcacagccgccctgggctgcctggtgaaggactacttccccgaaccggtgaccgtgtcctggaacagcggagccctgaccagcggcgtgcacaccttccccgccgtgctgcagagcagcggcctgtacagcctgagcagcgtggtgaccgtgcccagcagcagcctgggcacccagacctacatctgtaacgtgaaccacaagcccagcaacaccaaggtggacaagaaggtggagcccaagagctgtgacaagacccacacctgccccccctgccctgcccccgagctgctgggaggccccagcgtgttcctgttcccccccaagcctaaggacaccctgatgatcagcagaacccccgaggtgacctgtgtggtggtggatgtgagccacgaggaccctgaggtgaagttcaactggtacgtggacggcgtggaggtgcacaatgccaagaccaagcccagggaggagcagtacaacagcacctaccgggtggtgtccgtgctgaccgtgctgcaccaggattggctgaacggcaaggagtacaagtgtaaggtgtccaacaaggccctgcctgcccctatcgagaaaaccatcagcaaggccaagggccagcccagagagccccaggtgtacaccctgccccctagcagagatgagctgaccaagaaccaggtgtccctgacctgcctggtgaagggcttctaccccagcgacatcgccgtggagtgggagagcaacggccagcccgagaacaactacaagaccaccccccctgtgctggacagcgatggcagcttcttcctgtacagcaagctgaccgtggacaagagcagatggcagcagggcaacgtgttcagctgctccgtgatgcacgaggccctgcacaatcactacacccagaagagcctgagcctgtcccctggcaag

SEQ ID NO: 102 - protein, 445 aa, Artificial Sequence
  Humansed antibody sequence
QVQLVQSGAEVKKPGSSVKVSCKASGYTFTDYYMKWVRQAPGQGLEWMGEIYPNNGGITYNQKFKGRVTITADKSTSTAYMELSSLRSEDTAVYYCARGYEFVYWGQGTLVTVSSASTKGPSVFPLAPSSKSTSGGTAALGCLVKDYFPEPVTVSWNSGALTSGVHTFPAVLQSSGLYSLSSVVTVPSSSLGTQTYICNVNHKPSNTKVDKKVEPKSCDKTHTCPPCPAPELLGGPSVFLFPPKPKDTLMISRTPEVTCVVVDVSHEDPEVKFNWYVDGVEVHNAKTKPREEQYNSTYRVVSVLTVLHQDWLNGKEYKCKVSNKALPAPIEKTISKAKGQPREPQVYTLPPSRDELTKNQVSLTCLVKGFYPSDIAVEWESNGQPENNYKTTPPVLDSDGSFFLYSKLTVDKSRWQQGNVFSCSVMHEALHNHYTQKSLSLSPGK

SEQ ID NO: 103 - DNA, 1335 bp, Artificial Sequence
  Humansed antibody sequence
caggtgcagctggtgcagagcggcgccgaagtgaagaagcccggctccagcgtgaaggtgagctgcaaggctagcggctacaccttcaccgactactacatgaagtgggtgaggcaggcccccggccagggactggagtggatgggcgagatctaccccaacaacgggggcatcacctacaaccagaagttcaagggcagggtgaccatcaccgccgacaaaagcaccagcaccgcctacatggaactgagcagcctgaggagcgaggacaccgccgtgtactactgcgccaggggctacgagttcgtgtattggggccagggcacactagtgaccgtgtccagcgccagcaccaagggccccagcgtgttccccctggcccccagcagcaagagcaccagcggcggcacagccgccctgggctgcctggtgaaggactacttccccgaaccggtgaccgtgtcctggaacagcggagccctgaccagcggcgtgcacaccttccccgccgtgctgcagagcagcggcctgtacagcctgagcagcgtggtgaccgtgcccagcagcagcctgggcacccagacctacatctgtaacgtgaaccacaagcccagcaacaccaaggtggacaagaaggtggagcccaagagctgtgacaagacccacacctgccccccctgccctgcccccgagctgctgggaggccccagcgtgttcctgttcccccccaagcctaaggacaccctgatgatcagcagaacccccgaggtgacctgtgtggtggtggatgtgagccacgaggaccctgaggtgaagttcaactggtacgtggacggcgtggaggtgcacaatgccaagaccaagcccagggaggagcagtacaacagcacctaccgggtggtgtccgtgctgaccgtgctgcaccaggattggctgaacggcaaggagtacaagtgtaaggtgtccaacaaggccctgcctgcccctatcgagaaaaccatcagcaaggccaagggccagcccagagagccccaggtgtacaccctgccccctagcagagatgagctgaccaagaaccaggtgtccctgacctgcctggtgaagggcttctaccccagcgacatcgccgtggagtgggagagcaacggccagcccgagaacaactacaagaccaccccccctgtgctggacagcgatggcagcttcttcctgtacagcaagctgaccgtggacaagagcagatggcagcagggcaacgtgttcagctgctccgtgatgcacgaggccctgcacaatcactacacccagaagagcctgagcctgtcccctggcaag

SEQ ID NO: 104 - protein, 445 aa, Artificial Sequence
  Humansed antibody sequence
QVQLVQSGAEVKKPGSSVKVSCKASGYTFTDYYMKWVRQAPGQGLEWMGEIYPNNGGITYNQKFKGRVTITADKSTSTAYMELSSLRSEDTAVYYCANGYEFVYWGQGTLVTVSSASTKGPSVFPLAPSSKSTSGGTAALGCLVKDYFPEPVTVSWNSGALTSGVHTFPAVLQSSGLYSLSSVVTVPSSSLGTQTYICNVNHKPSNTKVDKKVEPKSCDKTHTCPPCPAPELLGGPSVFLFPPKPKDTLMISRTPEVTCVVVDVSHEDPEVKFNWYVDGVEVHNAKTKPREEQYNSTYRVVSVLTVLHQDWLNGKEYKCKVSNKALPAPIEKTISKAKGQPREPQVYTLPPSRDELTKNQVSLTCLVKGFYPSDIAVEWESNGQPENNYKTTPPVLDSDGSFFLYSKLTVDKSRWQQGNVFSCSVMHEALHNHYTQKSLSLSPGK

SEQ ID NO: 105 - DNA, 1335 bp, Artificial Sequence
  Humansed antibody sequence
caggtgcagctggtgcagagcggcgccgaagtgaagaagcccggctccagcgtgaaggtgagctgcaaggctagcggctacaccttcaccgactactacatgaagtgggtgaggcaggcccccggccagggactggagtggatgggcgagatctaccccaacaacgggggcatcacctacaaccagaagttcaagggcagggtgaccatcaccgccgacaaaagcaccagcaccgcctacatggaactgagcagcctgaggagcgaggacaccgccgtgtactactgcgccaacggctacgagttcgtgtattggggccagggcacactagtgaccgtgtccagcgccagcaccaagggccccagcgtgttccccctggcccccagcagcaagagcaccagcggcggcacagccgccctgggctgcctggtgaaggactacttccccgaaccggtgaccgtgtcctggaacagcggagccctgaccagcggcgtgcacaccttccccgccgtgctgcagagcagcggcctgtacagcctgagcagcgtggtgaccgtgcccagcagcagcctgggcacccagacctacatctgtaacgtgaaccacaagcccagcaacaccaaggtggacaagaaggtggagcccaagagctgtgacaagacccacacctgccccccctgccctgcccccgagctgctgggaggccccagcgtgttcctgttcccccccaagcctaaggacaccctgatgatcagcagaacccccgaggtgacctgtgtggtggtggatgtgagccacgaggaccctgaggtgaagttcaactggtacgtggacggcgtggaggtgcacaatgccaagaccaagcccagggaggagcagtacaacagcacctaccgggtggtgtccgtgctgaccgtgctgcaccaggattggctgaacggcaaggagtacaagtgtaaggtgtccaacaaggccctgcctgcccctatcgagaaaaccatcagcaaggccaagggccagcccagagagccccaggtgtacaccctgccccctagcagagatgagctgaccaagaaccaggtgtccctgacctgcctggtgaagggcttctaccccagcgacatcgccgtggagtgggagagcaacggccagcccgagaacaactacaagaccaccccccctgtgctggacagcgatggcagcttcttcctgtacagcaagctgaccgtggacaagagcagatggcagcagggcaacgtgttcagctgctccgtgatgcacgaggccctgcacaatcactacacccagaagagcctgagcctgtcccctggcaag

SEQ ID NO: 106 - protein, 445 aa, Artificial Sequence
  Humansed antibody sequence
QVQLVQSGAEVKKPGSSVKVSCKASGYTFTDYYMKWVRQAPGQGLEWIGEIYPNNGGITYNQKFKGRATLTVDKSTSTAYMELSSLRSEDTAVYYCANGYEFVYWGQGTLVTVSSASTKGPSVFPLAPSSKSTSGGTAALGCLVKDYFPEPVTVSWNSGALTSGVHTFPAVLQSSGLYSLSSVVTVPSSSLGTQTYICNVNHKPSNTKVDKKVEPKSCDKTHTCPPCPAPELLGGPSVFLFPPKPKDTLMISRTPEVTCVVVDVSHEDPEVKFNWYVDGVEVHNAKTKPREEQYNSTYRVVSVLTVLHQDWLNGKEYKCKVSNKALPAPIEKTISKAKGQPREPQVYTLPPSRDELTKNQVSLTCLVKGFYPSDIAVEWESNGQPENNYKTTPPVLDSDGSFFLYSKLTVDKSRWQQGNVFSCSVMHEALHNHYTQKSLSLSPGK

SEQ ID NO: 107 - DNA, 1335 bp, Artificial Sequence
  Humansed antibody sequence
caggtgcagctggtgcagagcggcgccgaagtgaagaagcccggctccagcgtgaaggtgagctgcaaggctagcggctacaccttcaccgactactacatgaagtgggtgaggcaggcccccggccagggactggagtggataggcgagatctaccccaacaacgggggcatcacctacaaccagaagttcaagggcagggcgaccctcaccgtcgacaaaagcaccagcaccgcctacatggaactgagcagcctgaggagcgaggacaccgccgtgtactactgcgccaacggctacgagttcgtgtattggggccagggcacactagtgaccgtgtccagcgccagcaccaagggccccagcgtgttccccctggcccccagcagcaagagcaccagcggcggcacagccgccctgggctgcctggtgaaggactacttccccgaaccggtgaccgtgtcctggaacagcggagccctgaccagcggcgtgcacaccttccccgccgtgctgcagagcagcggcctgtacagcctgagcagcgtggtgaccgtgcccagcagcagcctgggcacccagacctacatctgtaacgtgaaccacaagcccagcaacaccaaggtggacaagaaggtggagcccaagagctgtgacaagacccacacctgccccccctgccctgcccccgagctgctgggaggccccagcgtgttcctgttcccccccaagcctaaggacaccctgatgatcagcagaacccccgaggtgacctgtgtggtggtggatgtgagccacgaggaccctgaggtgaagttcaactggtacgtggacggcgtggaggtgcacaatgccaagaccaagcccagggaggagcagtacaacagcacctaccgggtggtgtccgtgctgaccgtgctgcaccaggattggctgaacggcaaggagtacaagtgtaaggtgtccaacaaggccctgcctgcccctatcgagaaaaccatcagcaaggccaagggccagcccagagagccccaggtgtacaccctgccccctagcagagatgagctgaccaagaaccaggtgtccctgacctgcctggtgaagggcttctaccccagcgacatcgccgtggagtgggagagcaacggccagcccgagaacaactacaagaccaccccccctgtgctggacagcgatggcagcttcttcctgtacagcaagctgaccgtggacaagagcagatggcagcagggcaacgtgttcagctgctccgtgatgcacgaggccctgcacaatcactacacccagaagagcctgagcctgtcccctggcaag

SEQ ID NO: 108 - protein, 445 aa, Artificial Sequence
  Humansed antibody sequence
QVQLVQSGAEVKKPGSSVKVSCKASGYTFTDYYMKWVRQAPGQGLEWMGEIYPNNGGITYNQKFKGRVTITADKSTSTAYMELSSLRSEDTAVYYCADGYEFVYWGQGTLVTVSSASTKGPSVFPLAPSSKSTSGGTAALGCLVKDYFPEPVTVSWNSGALTSGVHTFPAVLQSSGLYSLSSVVTVPSSSLGTQTYICNVNHKPSNTKVDKKVEPKSCDKTHTCPPCPAPELLGGPSVFLFPPKPKDTLMISRTPEVTCVVVDVSHEDPEVKFNWYVDGVEVHNAKTKPREEQYNSTYRVVSVLTVLHQDWLNGKEYKCKVSNKALPAPIEKTISKAKGQPREPQVYTLPPSRDELTKNQVSLTCLVKGFYPSDIAVEWESNGQPENNYKTTPPVLDSDGSFFLYSKLTVDKSRWQQGNVFSCSVMHEALHNHYTQKSLSLSPGK

SEQ ID NO: 109 - DNA, 1335 bp, Artificial Sequence
  Humansed antibody sequence
caggtgcagctggtgcagagcggcgccgaagtgaagaagcccggctccagcgtgaaggtgagctgcaaggctagcggctacaccttcaccgactactacatgaagtgggtgaggcaggcccccggccagggactggagtggatgggcgagatctaccccaacaacgggggcatcacctacaaccagaagttcaagggcagggtgaccatcaccgccgacaaaagcaccagcaccgcctacatggaactgagcagcctgaggagcgaggacaccgccgtgtactactgcgccgacggctacgagttcgtgtattggggccagggcacactagtgaccgtgtccagcgccagcaccaagggccccagcgtgttccccctggcccccagcagcaagagcaccagcggcggcacagccgccctgggctgcctggtgaaggactacttccccgaaccggtgaccgtgtcctggaacagcggagccctgaccagcggcgtgcacaccttccccgccgtgctgcagagcagcggcctgtacagcctgagcagcgtggtgaccgtgcccagcagcagcctgggcacccagacctacatctgtaacgtgaaccacaagcccagcaacaccaaggtggacaagaaggtggagcccaagagctgtgacaagacccacacctgccccccctgccctgcccccgagctgctgggaggccccagcgtgttcctgttcccccccaagcctaaggacaccctgatgatcagcagaacccccgaggtgacctgtgtggtggtggatgtgagccacgaggaccctgaggtgaagttcaactggtacgtggacggcgtggaggtgcacaatgccaagaccaagcccagggaggagcagtacaacagcacctaccgggtggtgtccgtgctgaccgtgctgcaccaggattggctgaacggcaaggagtacaagtgtaaggtgtccaacaaggccctgcctgcccctatcgagaaaaccatcagcaaggccaagggccagcccagagagccccaggtgtacaccctgccccctagcagagatgagctgaccaagaaccaggtgtccctgacctgcctggtgaagggcttctaccccagcgacatcgccgtggagtgggagagcaacggccagcccgagaacaactacaagaccaccccccctgtgctggacagcgatggcagcttcttcctgtacagcaagctgaccgtggacaagagcagatggcagcagggcaacgtgttcagctgctccgtgatgcacgaggccctgcacaatcactacacccagaagagcctgagcctgtcccctggcaag

SEQ ID NO: 110 - protein, 445 aa, Artificial Sequence
  Humansed antibody sequence
QVQLVQSGAEVKKPGSSVKVSCKASGYTFTDYYMKWVRQAPGQGLEWIGEIYPNNGGITYNQKFKGRATLTVDKSTSTAYMELSSLRSEDTAVYYCANGYEFDYWGQGTLVTVSSASTKGPSVFPLAPSSKSTSGGTAALGCLVKDYFPEPVTVSWNSGALTSGVHTFPAVLQSSGLYSLSSVVTVPSSSLGTQTYICNVNHKPSNTKVDKKVEPKSCDKTHTCPPCPAPELLGGPSVFLFPPKPKDTLMISRTPEVTCVVVDVSHEDPEVKFNWYVDGVEVHNAKTKPREEQYNSTYRVVSVLTVLHQDWLNGKEYKCKVSNKALPAPIEKTISKAKGQPREPQVYTLPPSRDELTKNQVSLTCLVKGFYPSDIAVEWESNGQPENNYKTTPPVLDSDGSFFLYSKLTVDKSRWQQGNVFSCSVMHEALHNHYTQKSLSLSPGK

SEQ ID NO: 111 - DNA, 1335 bp, Artificial Sequence
  Humansed antibody sequence
caggtgcagctggtgcagagcggcgccgaagtgaagaagcccggctccagcgtgaaggtgagctgcaaggctagcggctacaccttcaccgactactacatgaagtgggtgaggcaggcccccggccagggactggagtggataggcgagatctaccccaacaacgggggcatcacctacaaccagaagttcaagggcagggcgaccctcaccgtcgacaaaagcaccagcaccgcctacatggaactgagcagcctgaggagcgaggacaccgccgtgtactactgcgccaacggctacgagttcgactattggggccagggcacactagtgaccgtgtccagcgccagcaccaagggccccagcgtgttccccctggcccccagcagcaagagcaccagcggcggcacagccgccctgggctgcctggtgaaggactacttccccgaaccggtgaccgtgtcctggaacagcggagccctgaccagcggcgtgcacaccttccccgccgtgctgcagagcagcggcctgtacagcctgagcagcgtggtgaccgtgcccagcagcagcctgggcacccagacctacatctgtaacgtgaaccacaagcccagcaacaccaaggtggacaagaaggtggagcccaagagctgtgacaagacccacacctgccccccctgccctgcccccgagctgctgggaggccccagcgtgttcctgttcccccccaagcctaaggacaccctgatgatcagcagaacccccgaggtgacctgtgtggtggtggatgtgagccacgaggaccctgaggtgaagttcaactggtacgtggacggcgtggaggtgcacaatgccaagaccaagcccagggaggagcagtacaacagcacctaccgggtggtgtccgtgctgaccgtgctgcaccaggattggctgaacggcaaggagtacaagtgtaaggtgtccaacaaggccctgcctgcccctatcgagaaaaccatcagcaaggccaagggccagcccagagagccccaggtgtacaccctgccccctagcagagatgagctgaccaagaaccaggtgtccctgacctgcctggtgaagggcttctaccccagcgacatcgccgtggagtgggagagcaacggccagcccgagaacaactacaagaccaccccccctgtgctggacagcgatggcagcttcttcctgtacagcaagctgaccgtggacaagagcagatggcagcagggcaacgtgttcagctgctccgtgatgcacgaggccctgcacaatcactacacccagaagagcctgagcctgtcccctggcaag

SEQ ID NO: 112 - protein, 214 aa, Artificial Sequence
  Humansed antibody sequence
DIQMTQSPSSLSASVGDRVTITCSASQGISNYLNWYQQKPGKAPKLLIYYTSSLHSGVPSRFSGSGSGTDFTLTISSLQPEDFATYYCQQYSKLPWTFGQGTKLEIKRTVAAPSVFIFPPSDEQLKSGTASVVCLLNNFYPREAKVQWKVDNALQSGNSQESVTEQDSKDSTYSLSSTLTLSKADYEKHKVYACEVTHQGLSSPVTKSFNRGEC

SEQ ID NO: 113 - DNA, 642 bp, Artificial Sequence
  Humansed antibody sequence
gacatccagatgacccagagcccctcaagcctgagcgccagcgtgggcgacagggtgactatcacctgcagcgcctcccagggcatcagcaactacctgaactggtaccagcagaagcccggcaaggcccctaagctgctgatctactacaccagcagcctgcacagcggcgtgcccagcaggttctccggcagcggcagcggaaccgacttcaccctgaccattagcagcctccagcccgaggacttcgccacctactactgccagcagtacagcaagctgccctggaccttcggccagggcaccaaactggagatcaagcgtacggtggccgcccccagcgtgttcatcttcccccccagcgatgagcagctgaagagcggcaccgccagcgtggtgtgtctgctgaacaacttctacccccgggaggccaaggtgcagtggaaggtggacaatgccctgcagagcggcaacagccaggagagcgtgaccgagcaggacagcaaggactccacctacagcctgagcagcaccctgaccctgagcaaggccgactacgagaagcacaaggtgtacgcctgtgaggtgacccaccagggcctgtccagccccgtgaccaagagcttcaaccggggcgagtgc

SEQ ID NO: 114 - protein, 214 aa, Artificial Sequence
  Humansed antibody sequence
DIQMTQSPSSLSASVGDRVTITCSASQGISNYLNWYQQKPGKAPKLLIYYTSSLHSGVPSRFSGSGSGTDYTLTISSLQPEDFATYYCQQYSKLPWTFGQGTKLEIKRTVAAPSVFIFPPSDEQLKSGTASVVCLLNNFYPREAKVQWKVDNALQSGNSQESVTEQDSKDSTYSLSSTLTLSKADYEKHKVYACEVTHQGLSSPVTKSFNRGEC

SEQ ID NO: 115 - DNA, 642 bp, Artificial Sequence
  Humansed antibody sequence
gacatccagatgacccagagcccctcaagcctgagcgccagcgtgggcgacagggtgactatcacctgcagcgcctcccagggcatcagcaactacctgaactggtaccagcagaagcccggcaaggcccctaagctgctgatctactacaccagcagcctgcacagcggcgtgcccagcaggttctccggcagcggcagcggaaccgactacaccctgaccattagcagcctccagcccgaggacttcgccacctactactgccagcagtacagcaagctgccctggaccttcggccagggcaccaaactggagatcaagcgtacggtggccgcccccagcgtgttcatcttcccccccagcgatgagcagctgaagagcggcaccgccagcgtggtgtgtctgctgaacaacttctacccccgggaggccaaggtgcagtggaaggtggacaatgccctgcagagcggcaacagccaggagagcgtgaccgagcaggacagcaaggactccacctacagcctgagcagcaccctgaccctgagcaaggccgactacgagaagcacaaggtgtacgcctgtgaggtgacccaccagggcctgtccagccccgtgaccaagagcttcaaccggggcgagtgc

SEQ ID NO: 116 - protein, 118 aa, mus musculus
EVQLQQSGPVLVKPGASVKMSCEASGYTFTDYYMNWVKQSHGKTLEWIGVINPYNGGTDYNQKFKGKATLTVDKSSSTAYMELNSLTSEDSAVYYCARSVYDYPFDYWGQGTLVTVSS

SEQ ID NO: 117 - DNA, 354 bp, mus musculus
gaggtgcagctgcagcagagcggccccgtgctggtgaagcctggagccagcgtgaaaatgagctgcgaagccagcggctacaccttcaccgactactacatgaactgggtgaagcagagccacggcaagaccctggagtggatcggcgtgatcaacccctacaacgggggcaccgactacaaccagaagttcaagggcaaggccactctgaccgtggacaagagctccagcaccgcctacatggaactgaacagcctcacctctgaggacagcgccgtctattactgcgccaggagcgtgtacgactaccccttcgactactggggccagggcacactagtgaccgtgtccagc

SEQ ID NO: 118 - protein, 448 aa, Artificial Sequence
  Chimeric antibody sequence
EVQLQQSGPVLVKPGASVKMSCEASGYTFTDYYMNWVKQSHGKTLEWIGVINPYNGGTDYNQKFKGKATLTVDKSSSTAYMELNSLTSEDSAVYYCARSVYDYPFDYWGQGTLVTVSSASTKGPSVFPLAPSSKSTSGGTAALGCLVKDYFPEPVTVSWNSGALTSGVHTFPAVLQSSGLYSLSSVVTVPSSSLGTQTYICNVNHKPSNTKVDKKVEPKSCDKTHTCPPCPAPELLGGPSVFLFPPKPKDTLMISRTPEVTCVVVDVSHEDPEVKFNWYVDGVEVHNAKTKPREEQYNSTYRVVSVLTVLHQDWLNGKEYKCKVSNKALPAPIEKTISKAKGQPREPQVYTLPPSRDELTKNQVSLTCLVKGFYPSDIAVEWESNGQPENNYKTTPPVLDSDGSFFLYSKLTVDKSRWQQGNVFSCSVMHEALHNHYTQKSLSLSPGK

SEQ ID NO: 119 - DNA, 1344 bp, Artificial Sequence
  Chimeric antibody sequence
gaggtgcagctgcagcagagcggccccgtgctggtgaagcctggagccagcgtgaaaatgagctgcgaagccagcggctacaccttcaccgactactacatgaactgggtgaagcagagccacggcaagaccctggagtggatcggcgtgatcaacccctacaacgggggcaccgactacaaccagaagttcaagggcaaggccactctgaccgtggacaagagctccagcaccgcctacatggaactgaacagcctcacctctgaggacagcgccgtctattactgcgccaggagcgtgtacgactaccccttcgactactggggccagggcacactagtgaccgtgtccagcgccagcaccaagggccccagcgtgttccccctggcccccagcagcaagagcaccagcggcggcacagccgccctgggctgcctggtgaaggactacttccccgaaccggtgaccgtgtcctggaacagcggagccctgaccagcggcgtgcacaccttccccgccgtgctgcagagcagcggcctgtacagcctgagcagcgtggtgaccgtgcccagcagcagcctgggcacccagacctacatctgtaacgtgaaccacaagcccagcaacaccaaggtggacaagaaggtggagcccaagagctgtgacaagacccacacctgccccccctgccctgcccccgagctgctgggaggccccagcgtgttcctgttcccccccaagcctaaggacaccctgatgatcagcagaacccccgaggtgacctgtgtggtggtggatgtgagccacgaggaccctgaggtgaagttcaactggtacgtggacggcgtggaggtgcacaatgccaagaccaagcccagggaggagcagtacaacagcacctaccgggtggtgtccgtgctgaccgtgctgcaccaggattggctgaacggcaaggagtacaagtgtaaggtgtccaacaaggccctgcctgcccctatcgagaaaaccatcagcaaggccaagggccagcccagagagccccaggtgtacaccctgccccctagcagagatgagctgaccaagaaccaggtgtccctgacctgcctggtgaagggcttctaccccagcgacatcgccgtggagtgggagagcaacggccagcccgagaacaactacaagaccaccccccctgtgctggacagcgatggcagcttcttcctgtacagcaagctgaccgtggacaagagcagatggcagcagggcaacgtgttcagctgctccgtgatgcacgaggccctgcacaatcactacacccagaagagcctgagcctgtcccctggcaag

SEQ ID NO: 120 - protein, 111 aa, mus musculus
DIVLTQSPASLAVSLGQRATISCRASESVSIHGTHLMHWYQQKPGQPPKLLIYAASNLESGVPARFSGSGSETDFTLNIHPVEEEDAATYFCQQSIEDPRTFGGGTKLEIK

SEQ ID NO: 121 - DNA, 336 bp, mus musculus
gacatcgtcctgacccagagccccgccagcctggccgtgagcctgggccagagggccacaatcagctgcagggcctctgagtccgtgagcatccacggcacccacctgatgcactggtatcagcagaagcccggccagcctcccaagctgctgatctacgccgccagcaacctggagagcggcgtgcccgctaggttcagcggaagcggcagcgagaccgacttcaccctgaacatccaccccgtggaggaggaagacgccgccacctacttctgccagcagagcatcgaggaccccaggaccttcggcgggggcaccaagctcgagattaagcgt

SEQ ID NO: 122 - protein, 237 aa, Artificial Sequence
  Chimeric antibody sequence
MGWSCIILFLVATATGVHSDIVLTQSPASLAVSLGQRATISCRASESVSIHGTHLMHWYQQKPGQPPKLLIYAASNLESGVPARFSGSGSETDFTLNIHPVEEEDAATYFCQQSIEDPRTFGGGTKLEIKRTVAAPSVFIFPPSDEQLKSGTASVVCLLNNFYPREAKVQWKVDNALQSGNSQESVTEQDSKDSTYSLSSTLTLSKADYEKHKVYACEVTHQGLSSPVTKSFNRGEC

SEQ ID NO: 123 - DNA, 711 bp, Artificial Sequence
  Chimeric antibody sequence
atgggctggtcctgcatcatcctgtttctggtggccaccgccaccggcgtgcacagcgacatcgtcctgacccagagccccgccagcctggccgtgagcctgggccagagggccacaatcagctgcagggcctctgagtccgtgagcatccacggcacccacctgatgcactggtatcagcagaagcccggccagcctcccaagctgctgatctacgccgccagcaacctggagagcggcgtgcccgctaggttcagcggaagcggcagcgagaccgacttcaccctgaacatccaccccgtggaggaggaagacgccgccacctacttctgccagcagagcatcgaggaccccaggaccttcggcgggggcaccaagctcgagattaagcgtacggtggccgcccccagcgtgttcatcttcccccccagcgatgagcagctgaagagcggcaccgccagcgtggtgtgtctgctgaacaacttctacccccgggaggccaaggtgcagtggaaggtggacaatgccctgcagagcggcaacagccaggagagcgtgaccgagcaggacagcaaggactccacctacagcctgagcagcaccctgaccctgagcaaggccgactacgagaagcacaaggtgtacgcctgtgaggtgacccaccagggcctgtccagccccgtgaccaagagcttcaaccggggcgagtgc

SEQ ID NO: 124 - protein, 119 aa, mus musculus
EVQLQQSGPELVKPGTSVKIPCKTSGYIFTDYSIDWVKQSHGKSLEWIGDIDPNYGDPIYNHKFKGKATLTVDRSSSTAYMELRSLTSEDTAVYFCARRATGTDWFAFWGQGTLVTVSS

SEQ ID NO: 125 - DNA, 357 bp, mus musculus
gaggtgcagctgcagcagagcggccccgagctggtgaaacccggcaccagcgtgaagatcccctgcaagacctctggctacatcttcaccgactacagcatcgactgggtgaagcagagccacggcaagtctctggagtggattggggacatcgaccccaactacggcgaccccatctacaaccacaagttcaagggcaaggccaccctgaccgtggacaggagcagcagcaccgcctacatggaactcaggagcctgaccagcgaggacaccgccgtgtatttttgcgccaggagggccaccggcactgattggttcgccttctggggccagggcacactagtgaccgtgtccagc

SEQ ID NO: 126 - protein, 449 aa, Artificial Sequence
  Chimeric antibody sequence
EVQLQQSGPELVKPGTSVKIPCKTSGYIFTDYSIDWVKQSHGKSLEWIGDIDPNYGDPIYNHKFKGKATLTVDRSSSTAYMELRSLTSEDTAVYFCARRATGTDWFAFWGQGTLVTVSSASTKGPSVFPLAPSSKSTSGGTAALGCLVKDYFPEPVTVSWNSGALTSGVHTFPAVLQSSGLYSLSSVVTVPSSSLGTQTYICNVNHKPSNTKVDKKVEPKSCDKTHTCPPCPAPELLGGPSVFLFPPKPKDTLMISRTPEVTCVVVDVSHEDPEVKFNWYVDGVEVHNAKTKPREEQYNSTYRVVSVLTVLHQDWLNGKEYKCKVSNKALPAPIEKTISKAKGQPREPQVYTLPPSRDELTKNQVSLTCLVKGFYPSDIAVEWESNGQPENNYKTTPPVLDSDGSFFLYSKLTVDKSRWQQGNVFSCSVMHEALHNHYTQKSLSLSPGK

SEQ ID NO: 127 - DNA, 1347 bp, Artificial Sequence
  Chimeric antibody sequence
gaggtgcagctgcagcagagcggccccgagctggtgaaacccggcaccagcgtgaagatcccctgcaagacctctggctacatcttcaccgactacagcatcgactgggtgaagcagagccacggcaagtctctggagtggattggggacatcgaccccaactacggcgaccccatctacaaccacaagttcaagggcaaggccaccctgaccgtggacaggagcagcagcaccgcctacatggaactcaggagcctgaccagcgaggacaccgccgtgtatttttgcgccaggagggccaccggcactgattggttcgccttctggggccagggcacactagtgaccgtgtccagcgccagcaccaagggccccagcgtgttccccctggcccccagcagcaagagcaccagcggcggcacagccgccctgggctgcctggtgaaggactacttccccgaaccggtgaccgtgtcctggaacagcggagccctgaccagcggcgtgcacaccttccccgccgtgctgcagagcagcggcctgtacagcctgagcagcgtggtgaccgtgcccagcagcagcctgggcacccagacctacatctgtaacgtgaaccacaagcccagcaacaccaaggtggacaagaaggtggagcccaagagctgtgacaagacccacacctgccccccctgccctgcccccgagctgctgggaggccccagcgtgttcctgttcccccccaagcctaaggacaccctgatgatcagcagaacccccgaggtgacctgtgtggtggtggatgtgagccacgaggaccctgaggtgaagttcaactggtacgtggacggcgtggaggtgcacaatgccaagaccaagcccagggaggagcagtacaacagcacctaccgggtggtgtccgtgctgaccgtgctgcaccaggattggctgaacggcaaggagtacaagtgtaaggtgtccaacaaggccctgcctgcccctatcgagaaaaccatcagcaaggccaagggccagcccagagagccccaggtgtacaccctgccccctagcagagatgagctgaccaagaaccaggtgtccctgacctgcctggtgaagggcttctaccccagcgacatcgccgtggagtgggagagcaacggccagcccgagaacaactacaagaccaccccccctgtgctggacagcgatggcagcttcttcctgtacagcaagctgaccgtggacaagagcagatggcagcagggcaacgtgttcagctgctccgtgatgcacgaggccctgcacaatcactacacccagaagagcctgagcctgtcccctggcaag

SEQ ID NO: 128 - protein, 108 aa, mus musculus
DIQMTQSPASLSVSVGETVTITCRASENIYNNLAWYQQKQGKSPQLLVYAATILADGVPSRFSGSGSGTQYSLKINSLQSGDFGTYYCQHFWGTPLTFGAGTKLELKR

SEQ ID NO: 129 - DNA, 324 bp, mus musculus
gacatccagatgacccagagccccgctagcctcagcgtgtccgtcggcgagaccgtgaccatcacctgcagggccagcgagaacatctacaacaacctggcctggtatcagcagaagcagggcaaaagcccccagctgctggtgtacgccgccaccattctggccgacggcgtgcccagcaggttctctggaagcggcagcggcacccagtacagcctgaagatcaacagcctgcagagcggggacttcggcacctactactgccagcacttctggggcactcccctgaccttcggagccggcaccaagctggagctgaagcgt

SEQ ID NO: 130 - protein, 214 aa, Artificial Sequence
  Chimeric antibody sequence
DIQMTQSPASLSVSVGETVTITCRASENIYNNLAWYQQKQGKSPQLLVYAATILADGVPSRFSGSGSGTQYSLKINSLQSGDFGTYYCQHFWGTPLTFGAGTKLELKRTVAAPSVFIFPPSDEQLKSGTASVVCLLNNFYPREAKVQWKVDNALQSGNSQESVTEQDSKDSTYSLSSTLTLSKADYEKHKVYACEVTHQGLSSPVTKSFNRGEC

SEQ ID NO: 131 - DNA, 642 bp, Artificial Sequence
  Chimeric antibody sequence
gacatccagatgacccagagccccgctagcctcagcgtgtccgtcggcgagaccgtgaccatcacctgcagggccagcgagaacatctacaacaacctggcctggtatcagcagaagcagggcaaaagcccccagctgctggtgtacgccgccaccattctggccgacggcgtgcccagcaggttctctggaagcggcagcggcacccagtacagcctgaagatcaacagcctgcagagcggggacttcggcacctactactgccagcacttctggggcactcccctgaccttcggagccggcaccaagctggagctgaagcgtacggtggccgcccccagcgtgttcatcttcccccccagcgatgagcagctgaagagcggcaccgccagcgtggtgtgtctgctgaacaacttctacccccgggaggccaaggtgcagtggaaggtggacaatgccctgcagagcggcaacagccaggagagcgtgaccgagcaggacagcaaggactccacctacagcctgagcagcaccctgaccctgagcaaggccgactacgagaagcacaaggtgtacgcctgtgaggtgacccaccagggcctgtccagccccgtgaccaagagcttcaaccggggcgagtgc

SEQ ID NO: 132 - protein, 118 aa, mus musculus
QVQLQQPGAELVKPGASVKLSCKASGYTFTNYWMHWVKQRPGQGLEWIGIIHPNSGSTNYNEKFKSKATLTVDKSSSTAYMQLSSLTSEDSAVYYCARGIYDYPFAYWGQGTLVTVSS

SEQ ID NO: 133 - DNA, 354 bp, mus musculus
caggtgcagctccagcagcccggagccgaactggtgaagcccggagccagcgtcaaactgtcctgcaaggccagcggctacaccttcaccaactactggatgcactgggtgaagcagaggcccggccagggcctggagtggatcggcatcatccaccccaacagcgggagcaccaactacaacgagaagttcaagagcaaggccaccctgaccgtggacaagagcagcagcactgcctacatgcagctgagcagcctgaccagcgaggacagcgctgtgtactactgcgccaggggcatctacgactaccccttcgcctattggggccagggcacactagtgaccgtgtccagc

SEQ ID NO: 134 - protein, 448 aa, Artificial Sequence
  Chimeric antibody sequence
QVQLQQPGAELVKPGASVKLSCKASGYTFTNYWMHWVKQRPGQGLEWIGIIHPNSGSTNYNEKFKSKATLTVDKSSSTAYMQLSSLTSEDSAVYYCARGIYDYPFAYWGQGTLVTVSSASTKGPSVFPLAPSSKSTSGGTAALGCLVKDYFPEPVTVSWNSGALTSGVHTFPAVLQSSGLYSLSSVVTVPSSSLGTQTYICNVNHKPSNTKVDKKVEPKSCDKTHTCPPCPAPELLGGPSVFLFPPKPKDTLMISRTPEVTCVVVDVSHEDPEVKFNWYVDGVEVHNAKTKPREEQYNSTYRVVSVLTVLHQDWLNGKEYKCKVSNKALPAPIEKTISKAKGQPREPQVYTLPPSRDELTKNQVSLTCLVKGFYPSDIAVEWESNGQPENNYKTTPPVLDSDGSFFLYSKLTVDKSRWQQGNVFSCSVMHEALHNHYTQKSLSLSPGK

SEQ ID NO: 135 - DNA, 1344 bp, Artificial Sequence
  Chimeric antibody sequence
caggtgcagctccagcagcccggagccgaactggtgaagcccggagccagcgtcaaactgtcctgcaaggccagcggctacaccttcaccaactactggatgcactgggtgaagcagaggcccggccagggcctggagtggatcggcatcatccaccccaacagcgggagcaccaactacaacgagaagttcaagagcaaggccaccctgaccgtggacaagagcagcagcactgcctacatgcagctgagcagcctgaccagcgaggacagcgctgtgtactactgcgccaggggcatctacgactaccccttcgcctattggggccagggcacactagtgaccgtgtccagcgccagcaccaagggccccagcgtgttccccctggcccccagcagcaagagcaccagcggcggcacagccgccctgggctgcctggtgaaggactacttccccgaaccggtgaccgtgtcctggaacagcggagccctgaccagcggcgtgcacaccttccccgccgtgctgcagagcagcggcctgtacagcctgagcagcgtggtgaccgtgcccagcagcagcctgggcacccagacctacatctgtaacgtgaaccacaagcccagcaacaccaaggtggacaagaaggtggagcccaagagctgtgacaagacccacacctgccccccctgccctgcccccgagctgctgggaggccccagcgtgttcctgttcccccccaagcctaaggacaccctgatgatcagcagaacccccgaggtgacctgtgtggtggtggatgtgagccacgaggaccctgaggtgaagttcaactggtacgtggacggcgtggaggtgcacaatgccaagaccaagcccagggaggagcagtacaacagcacctaccgggtggtgtccgtgctgaccgtgctgcaccaggattggctgaacggcaaggagtacaagtgtaaggtgtccaacaaggccctgcctgcccctatcgagaaaaccatcagcaaggccaagggccagcccagagagccccaggtgtacaccctgccccctagcagagatgagctgaccaagaaccaggtgtccctgacctgcctggtgaagggcttctaccccagcgacatcgccgtggagtgggagagcaacggccagcccgagaacaactacaagaccaccccccctgtgctggacagcgatggcagcttcttcctgtacagcaagctgaccgtggacaagagcagatggcagcagggcaacgtgttcagctgctccgtgatgcacgaggccctgcacaatcactacacccagaagagcctgagcctgtcccctggcaag

SEQ ID NO: 136 - protein, 112 aa, mus musculus
DIVLTQSPASLAVSLGQRATISCRASESVSIHGTHLMHWYQQKPGQPPKLLIYAASNLESGVPARFSGSGSETDFTLNIHPVEEEDAATYFCQQSIEDPYTFGGGTKLEIKR

SEQ ID NO: 137 - DNA, 336 bp, mus musculus
gacatcgtgctgacccagtctcccgctagcctggccgtgtctctgggccagagggccacaatcagctgcagggccagcgagagcgtcagcattcacggcacccacctgatgcactggtaccagcagaagcccggccagcctcccaagctcctgatctacgccgccagcaacctggaaagcggagtgcccgccaggttcagcggcagcggctccgagaccgacttcaccctgaacatccaccccgtggaggaggaggacgccgccacctacttctgccagcagagcatcgaggacccctacaccttcggcggcggcaccaagctggagatcaagcgt

SEQ ID NO: 138 - protein, 218 aa, Artificial Sequence
  Chimeric antibody sequence
DIVLTQSPASLAVSLGQRATISCRASESVSIHGTHLMHWYQQKPGQPPKLLIYAASNLESGVPARFSGSGSETDFTLNIHPVEEEDAATYFCQQSIEDPYTFGGGTKLEIKRTVAAPSVFIFPPSDEQLKSGTASVVCLLNNFYPREAKVQWKVDNALQSGNSQESVTEQDSKDSTYSLSSTLTLSKADYEKHKVYACEVTHQGLSSPVTKSFNRGEC

SEQ ID NO: 139 - DNA, 654 bp, Artificial Sequence
  Chimeric antibody sequence
gacatcgtgctgacccagtctcccgctagcctggccgtgtctctgggccagagggccacaatcagctgcagggccagcgagagcgtcagcattcacggcacccacctgatgcactggtaccagcagaagcccggccagcctcccaagctcctgatctacgccgccagcaacctggaaagcggagtgcccgccaggttcagcggcagcggctccgagaccgacttcaccctgaacatccaccccgtggaggaggaggacgccgccacctacttctgccagcagagcatcgaggacccctacaccttcggcggcggcaccaagctggagatcaagcgtacggtggccgcccccagcgtgttcatcttcccccccagcgatgagcagctgaagagcggcaccgccagcgtggtgtgtctgctgaacaacttctacccccgggaggccaaggtgcagtggaaggtggacaatgccctgcagagcggcaacagccaggagagcgtgaccgagcaggacagcaaggactccacctacagcctgagcagcaccctgaccctgagcaaggccgactacgagaagcacaaggtgtacgcctgtgaggtgacccaccagggcctgtccagccccgtgaccaagagcttcaaccggggcgagtgc

SEQ ID NO: 140 - protein, 120 aa, mus musculus
EVKLLQSGGGLVQPGGSLKLSCAASGIDFSRYWMSWVRRAPGKGLEWIGEINPDRSTINYAPSLKDKFIISRDNAKNTLYLQMSKVRSEDTALYYCAVFYYDYEGAMDYWGQGTSVTVSS

SEQ ID NO: 141 - DNA, 360 bp, mus musculus
gaggtgaagcttctccagtctggaggtggcctggtgcagcctggaggatccctgaaactctcctgtgcagcctcaggaatcgattttagtagatactggatgagttgggttcggcgggctccagggaaaggactagaatggattggagaaattaatccagataggagtacaatcaactatgcaccatctctaaaggataaattcatcatctccagagacaacgccaaaaatacgctgtacctgcaaatgagcaaagtgagatctgaggacacagccctttattactgtgcagttttctactatgattacgagggtgctatggactactggggtcaaggaacctcagtcaccgtctcctca

SEQ ID NO: 142 - protein, 450 aa, Artificial Sequence
  Chimeric antibody sequence
EVKLLQSGGGLVQPGGSLKLSCAASGIDFSRYWMSWVRRAPGKGLEWIGEINPDRSTINYAPSLKDKFIISRDNAKNTLYLQMSKVRSEDTALYYCAVFYYDYEGAMDYWGQGTSVTVSSAKTTAPSVFPLAPSSKSTSGGTAALGCLVKDYFPEPVTVSWNSGALTSGVHTFPAVLQSSGLYSLSSVVTVPSSSLGTQTYICNVNHKPSNTKVDKKVEPKSCDKTHTCPPCPAPELLGGPSVFLFPPKPKDTLMISRTPEVTCVVVDVSHEDPEVKFNWYVDGVEVHNAKTKPREEQYNSTYRVVSVLTVLHQDWLNGKEYKCKVSNKALPAPIEKTISKAKGQPREPQVYTLPPSRDELTKNQVSLTCLVKGFYPSDIAVEWESNGQPENNYKTTPPVLDSDGSFFLYSKLTVDKSRWQQGNVFSCSVMHEALHNHYTQKSLSLSPGK

SEQ ID NO: 143 - DNA, 1350 bp, Artificial Sequence
  Chimeric antibody sequence
gaggtgaagcttctccagtctggaggtggcctggtgcagcctggaggatccctgaaactctcctgtgcagcctcaggaatcgattttagtagatactggatgagttgggttcggcgggctccagggaaaggactagaatggattggagaaattaatccagataggagtacaatcaactatgcaccatctctaaaggataaattcatcatctccagagacaacgccaaaaatacgctgtacctgcaaatgagcaaagtgagatctgaggacacagccctttattactgtgcagttttctactatgattacgagggtgctatggactactggggtcaaggaacctcagtcaccgtctcctcagccaaaacaacagcccccagcgtgttccccctggcccccagcagcaagagcaccagcggcggcacagccgccctgggctgcctggtgaaggactacttccccgaaccggtgaccgtgtcctggaacagcggagccctgaccagcggcgtgcacaccttccccgccgtgctgcagagcagcggcctgtacagcctgagcagcgtggtgaccgtgcccagcagcagcctgggcacccagacctacatctgtaacgtgaaccacaagcccagcaacaccaaggtggacaagaaggtggagcccaagagctgtgacaagacccacacctgccccccctgccctgcccccgagctgctgggaggccccagcgtgttcctgttcccccccaagcctaaggacaccctgatgatcagcagaacccccgaggtgacctgtgtggtggtggatgtgagccacgaggaccctgaggtgaagttcaactggtacgtggacggcgtggaggtgcacaatgccaagaccaagcccagggaggagcagtacaacagcacctaccgggtggtgtccgtgctgaccgtgctgcaccaggattggctgaacggcaaggagtacaagtgtaaggtgtccaacaaggccctgcctgcccctatcgagaaaaccatcagcaaggccaagggccagcccagagagccccaggtgtacaccctgccccctagcagagatgagctgaccaagaaccaggtgtccctgacctgcctggtgaagggcttctaccccagcgacatcgccgtggagtgggagagcaacggccagcccgagaacaactacaagaccaccccccctgtgctggacagcgatggcagcttcttcctgtacagcaagctgaccgtggacaagagcagatggcagcagggcaacgtgttcagctgctccgtgatgcacgaggccctgcacaatcactacacccagaagagcctgagcctgtcccctggcaag

SEQ ID NO: 144 - protein, 108 aa, mus musculus
DIVMTQSQKFMSTSVGDRVSVTCKASQNVDTNVAWYQQKPGQSPKALIYSASYRFSGVPDRFTGSGSGTDFTLTISNVQSEDLAEYFCQQYNSFPFTFGSGTKLEIKR

SEQ ID NO: 145 - DNA, 324 bp, mus musculus
gacattgtgatgacccagtctcaaaaattcatgtccacatcagtaggagacagggtcagcgtcacctgcaaggccagtcagaatgtggatactaatgtagcctggtatcaacaaaaaccagggcaatctcctaaagcactgatttactcggcatcctaccggttcagtggagtccctgatcgcttcacaggcagtggatctgggacagatttcactctcaccatcagcaatgtgcagtctgaagacttggcagagtatttctgtcagcaatataacagctttccattcacgttcggctcggggacaaagttggaaataaaacgt

SEQ ID NO: 146 - protein, 214 aa, Artificial Sequence
  Chimeric antibody sequence
DIVMTQSQKFMSTSVGDRVSVTCKASQNVDTNVAWYQQKPGQSPKALIYSASYRFSGVPDRFTGSGSGTDFTLTISNVQSEDLAEYFCQQYNSFPFTFGSGTKLEIKRTVAAPSVFIFPPSDEQLKSGTASVVCLLNNFYPREAKVQWKVDNALQSGNSQESVTEQDSKDSTYSLSSTLTLSKADYEKHKVYACEVTHQGLSSPVTKSFNRGEC

SEQ ID NO: 147 - protein, 642 aa, Artificial Sequence
  Chimeric antibody sequence
GACATTGTGATGACCCAGTCTCAAAAATTCATGTCCACATCAGTAGGAGACAGGGTCAGCGTCACCTGCAAGGCCAGTCAGAATGTGGATACTAATGTAGCCTGGTATCAACAAAAACCAGGGCAATCTCCTAAAGCACTGATTTACTCGGCATCCTACCGGTTCAGTGGAGTCCCTGATCGCTTCACAGGCAGTGGATCTGGGACAGATTTCACTCTCACCATCAGCAATGTGCAGTCTGAAGACTTGGCAGAGTATTTCTGTCAGCAATATAACAGCTTTCCATTCACGTTCGGCTCGGGGACAAAGTTGGAAATAAAACGTACGGTGGCCGCCCCCAGCGTGTTCATCTTCCCCCCCAGCGATGAGCAGCTGAAGAGCGGCACCGCCAGCGTGGTGTGTCTGCTGAACAACTTCTACCCCCGGGAGGCCAAGGTGCAGTGGAAGGTGGACAATGCCCTGCAGAGCGGCAACAGCCAGGAGAGCGTGACCGAGCAGGACAGCAAGGACTCCACCTACAGCCTGAGCAGCACCCTGACCCTGAGCAAGGCCGACTACGAGAAGCACAAGGTGTACGCCTGTGAGGTGACCCACCAGGGCCTGTCCAGCCCCGTGACCAAGAGCTTCAACCGGGGCGAGTGC

SEQ ID NO: 148 - protein, 118 aa, mus musculus
PVQLQQPGTELVRPGTSVKLSCKASGYTFTSYWMHWVKQRPGQGLEWIGVIDPSDSYTNYNQKFKGKATLTVDTSSSTAYMQLSSLTSEDSAVYYCARQVFDYPMDYWGQGTSVTVSS

SEQ ID NO: 149 - DNA, 354 bp, mus musculus
ccggtccaactgcagcagcctgggactgagctggtgaggcctgggacttcagtgaagttgtcctgcaaggcttctggctacaccttcaccagctactggatgcactgggtaaagcagaggcctggacaaggccttgagtggatcggagtgattgatccttctgatagttatactaactacaatcaaaagttcaagggcaaggccacattgactgtagacacatcctccagcacagcctacatgcagctcagcagcctgacatctgaggactctgcggtctattactgtgcaagacaggtgtttgactatcctatggactactggggtcaaggaacctcagtcaccgtctcctca

SEQ ID NO: 150 - protein, 448 aa, Artificial Sequence
  Chimeric antibody sequence
PVQLQQPGTELVRPGTSVKLSCKASGYTFTSHWMHWVKQRPGQGLEWIGVIDPSDSYTNYNQKFKGKATLTVDTSSSTAYMQLSSLTSEDSAVYYCARQVFDYPMDYWGQGTLVTVSSASTKGPSVFPLAPSSKSTSGGTAALGCLVKDYFPEPVTVSWNSGALTSGVHTFPAVLQSSGLYSLSSVVTVPSSSLGTQTYICNVNHKPSNTKVDKKVEPKSCDKTHTCPPCPAPELLGGPSVFLFPPKPKDTLMISRTPEVTCVVVDVSHEDPEVKFNWYVDGVEVHNAKTKPREEQYNSTYRVVSVLTVLHQDWLNGKEYKCKVSNKALPAPIEKTISKAKGQPREPQVYTLPPSRDELTKNQVSLTCLVKGFYPSDIAVEWESNGQPENNYKTTPPVLDSDGSFFLYSKLTVDKSRWQQGNVFSCSVMHEALHNHYTQKSLSLSPGK

SEQ ID NO: 151 - DNA, 1344 bp, Artificial Sequence
  Chimeric antibody sequence
ccggtccaactgcagcagcctgggactgagctggtgaggcctgggacttcagtgaagttgtcctgcaaggcttctggctacaccttcaccagccactggatgcactgggtaaagcagaggcctggacaaggccttgagtggatcggagtgattgatccttctgatagttatactaactacaatcaaaagttcaagggcaaggccacattgactgtagacacatcctccagcacagcctacatgcagctcagcagcctgacatctgaggactctgcggtctattactgtgcaagacaggtgtttgactatcctatggactactggggtcaaggaacactagtgaccgtgtccagcgccagcaccaagggccccagcgtgttccccctggcccccagcagcaagagcaccagcggcggcacagccgccctgggctgcctggtgaaggactacttccccgaaccggtgaccgtgtcctggaacagcggagccctgaccagcggcgtgcacaccttccccgccgtgctgcagagcagcggcctgtacagcctgagcagcgtggtgaccgtgcccagcagcagcctgggcacccagacctacatctgtaacgtgaaccacaagcccagcaacaccaaggtggacaagaaggtggagcccaagagctgtgacaagacccacacctgccccccctgccctgcccccgagctgctgggaggccccagcgtgttcctgttcccccccaagcctaaggacaccctgatgatcagcagaacccccgaggtgacctgtgtggtggtggatgtgagccacgaggaccctgaggtgaagttcaactggtacgtggacggcgtggaggtgcacaatgccaagaccaagcccagggaggagcagtacaacagcacctaccgggtggtgtccgtgctgaccgtgctgcaccaggattggctgaacggcaaggagtacaagtgtaaggtgtccaacaaggccctgcctgcccctatcgagaaaaccatcagcaaggccaagggccagcccagagagccccaggtgtacaccctgccccctagcagagatgagctgaccaagaaccaggtgtccctgacctgcctggtgaagggcttctaccccagcgacatcgccgtggagtgggagagcaacggccagcccgagaacaactacaagaccaccccccctgtgctggacagcgatggcagcttcttcctgtacagcaagctgaccgtggacaagagcagatggcagcagggcaacgtgttcagctgctccgtgatgcacgaggccctgcacaatcactacacccagaagagcctgagcctgtcccctggcaag

SEQ ID NO: 152 - protein, 112 aa, mus musculus
DIVLTQSPASLAVSLGQRATISCRASESVSIHGTHLMHWYQQKPGQPPKLLIYAASNLESGVPARFSGSGSETDFTLNIHPVEEEDAATYFCQQSIEDPWTFGGGTKLEIKR

SEQ ID NO: 153 - DNA, 336 bp, mus musculus
gacattgtgctgacccaatctccagcttctttggctgtgtctctagggcagagggccaccatctcctgcagagccagtgaaagtgtcagtattcatggtactcatttaatgcactggtaccaacagaaaccaggacagccacccaaactcctcatctatgctgcatccaacctagaatctggagtccctgccaggttcagtggcagtgggtctgagacagacttcaccctcaacatccatcctgtggaggaggaggatgctgcaacctatttctgtcagcaaagtattgaggatccgtggacgttcggtggaggcaccaagctggaaatcaaacgt

SEQ ID NO: 154 - protein, 218 aa, Artificial Sequence
  Chimeric antibody sequence
DIVLTQSPASLAVSLGQRATISCRASESVSIHGTHLMHWYQQKPGQPPKLLIYAASNLESGVPARFSGSGSETDFTLNIHPVEEEDAATYFCQQSIEDPWTFGGGTKLEINRTVAAPSVFIFPPSDEQLKSGTASVVCLLNNFYPREAKVQWKVDNALQSGNSQESVTEQDSKDSTYSLSSTLTLSKADYEKHKVYACEVTHQGLSSPVTKSFNRGEC

SEQ ID NO: 155 - DNA, 654 bp, Artificial Sequence
  Chimeric antibody sequence
gacattgtgctgacccaatctccagcttctttggctgtgtctctagggcagagggccaccatctcctgcagagccagtgaaagtgtcagtattcatggtactcatttaatgcactggtaccaacagaaaccaggacagccacccaaactcctcatctatgctgcatccaacctagaatctggagtccctgccaggttcagtggcagtgggtctgagacagacttcaccctcaacatccatcctgtggaggaggaggatgctgcaacctatttctgtcagcaaagtattgaggatccgtggacgttcggtggaggcaccaagctggaaatcaatcgtacggtggccgcccccagcgtgttcatcttcccccccagcgatgagcagctgaagagcggcaccgccagcgtggtgtgtctgctgaacaacttctacccccgggaggccaaggtgcagtggaaggtggacaatgccctgcagagcggcaacagccaggagagcgtgaccgagcaggacagcaaggactccacctacagcctgagcagcaccctgaccctgagcaaggccgactacgagaagcacaaggtgtacgcctgtgaggtgacccaccagggcctgtccagccccgtgaccaagagcttcaaccggggcgagtgc

SEQ ID NO: 156 - protein, 118 aa, mus musculus
QVQLQQSGAELVRPGASVTLSCKASGYTFTDYEMHWVKQTPVHGLEWIGAIDPETGGTAYNQKFKGKAILTADKSSSTAYMELRSLTSEDSAVYYCTRSIYDYYFDYWGQGTTLTVSS

SEQ ID NO: 157 - DNA, 354 bp, mus musculus
caggttcaactgcagcagtctggggctgagctggtgaggcctggggcttcagtgacgctgtcctgcaaggcttcgggctacacatttactgactatgaaatgcactgggtgaagcagacacctgtgcatggcctggaatggattggagctattgatcctgaaactggtggtactgcctacaatcagaagttcaagggcaaggccatactgactgcagacaaatcctccagcacagcctacatggagctccgcagcctgacatctgaggactctgccgtctattactgtacaagatcgatttatgattactactttgactactggggccaaggcaccactctcacagtctcctca

SEQ ID NO: 158 - protein, 448 aa, Artificial Sequence
  Chimeric antibody sequence
QVQLQQSGAELVRPGASVTLSCKASGYTFTDYEMHWVKQTPVHGLEWIGAIDPETGGTAYNQKFKGKAILTADKSSSTAYMELRSLTSEDSAVYYCTRSIYDYYFDYWGQGTTLTVSSAKTTPPSVFPLAPSSKSTSGGTAALGCLVKDYFPEPVTVSWNSGALTSGVHTFPAVLQSSGLYSLSSVVTVPSSSLGTQTYICNVNHKPSNTKVDKKVEPKSCDKTHTCPPCPAPELLGGPSVFLFPPKPKDTLMISRTPEVTCVVVDVSHEDPEVKFNWYVDGVEVHNAKTKPREEQYNSTYRVVSVLTVLHQDWLNGKEYKCKVSNKALPAPIEKTISKAKGQPREPQVYTLPPSRDELTKNQVSLTCLVKGFYPSDIAVEWESNGQPENNYKTTPPVLDSDGSFFLYSKLTVDKSRWQQGNVFSCSVMHEALHNHYTQKSLSLSPGK

SEQ ID NO: 159 - DNA, 1344 bp, Artificial Sequence
  Chimeric antibody sequence
caggttcaactgcagcagtctggggctgagctggtgaggcctggggcttcagtgacgctgtcctgcaaggcttcgggctacacatttactgactatgaaatgcactgggtgaagcagacacctgtgcatggcctggaatggattggagctattgatcctgaaactggtggtactgcctacaatcagaagttcaagggcaaggccatactgactgcagacaaatcctccagcacagcctacatggagctccgcagcctgacatctgaggactctgccgtctattactgtacaagatcgatttatgattactactttgactactggggccaaggcaccactctcacagtctcctcagccaaaacgacaccccccagcgtgttccccctggcccccagcagcaagagcaccagcggcggcacagccgccctgggctgcctggtgaaggactacttccccgaaccggtgaccgtgtcctggaacagcggagccctgaccagcggcgtgcacaccttccccgccgtgctgcagagcagcggcctgtacagcctgagcagcgtggtgaccgtgcccagcagcagcctgggcacccagacctacatctgtaacgtgaaccacaagcccagcaacaccaaggtggacaagaaggtggagcccaagagctgtgacaagacccacacctgccccccctgccctgcccccgagctgctgggaggccccagcgtgttcctgttcccccccaagcctaaggacaccctgatgatcagcagaacccccgaggtgacctgtgtggtggtggatgtgagccacgaggaccctgaggtgaagttcaactggtacgtggacggcgtggaggtgcacaatgccaagaccaagcccagggaggagcagtacaacagcacctaccgggtggtgtccgtgctgaccgtgctgcaccaggattggctgaacggcaaggagtacaagtgtaaggtgtccaacaaggccctgcctgcccctatcgagaaaaccatcagcaaggccaagggccagcccagagagccccaggtgtacaccctgccccctagcagagatgagctgaccaagaaccaggtgtccctgacctgcctggtgaagggcttctaccccagcgacatcgccgtggagtgggagagcaacggccagcccgagaacaactacaagaccaccccccctgtgctggacagcgatggcagcttcttcctgtacagcaagctgaccgtggacaagagcagatggcagcagggcaacgtgttcagctgctccgtgatgcacgaggccctgcacaatcactacacccagaagagcctgagcctgtcccctggcaag

SEQ ID NO: 160 - protein, 112 aa, mus musculus
DIVLTQSPASLAVSLGQRATISCRASESVSIHGTHLMHWYQQKPGQPPKLLIYAASNLESGVPARFSGGGSETDFTLNIHPVEEEDGATYFCQQSIEYPRTFGGGTKLEINR

SEQ ID NO: 161 - DNA, 336 bp, mus musculus
gacattgtgctgacccaatctccagcttctttggctgtgtctctagggcagagggccaccatctcctgcagagccagtgaaagtgtcagtattcatggtactcatttaatgcactggtaccaacagaaaccaggacagccacccaaactcctcatctatgctgcatccaacctagaatctggagtccctgccaggttcagtggcggtgggtctgagacagacttcaccctcaacatccatcctgtggaggaggaggatggtgcaacctatttctgtcagcaaagtattgagtatcctcggacgttcggtggaggcaccaagctggaaatcaatcgt

SEQ ID NO: 162 - protein, 218 aa, Artificial Sequence
  Chimeric antibody sequence
DIVLTQSPASLAVSLGQRATISCRASESVSIHGTHLMHWYQQKPGQPPKLLIYAASNLESGVPARFSGGGSETDFTLNIHPVEEEDGATYFCQQSIEYPRTFGGGTKLEINRTVAAPSVFIFPPSDEQLKSGTASVVCLLNNFYPREAKVQWKVDNALQSGNSQESVTEQDSKDSTYSLSSTLTLSKADYEKHKVYACEVTHQGLSSPVTKSFNRGEC

SEQ ID NO: 163 - DNA, 654 bp, Artificial Sequence
  Chimeric antibody sequence
gacattgtgctgacccaatctccagcttctttggctgtgtctctagggcagagggccaccatctcctgcagagccagtgaaagtgtcagtattcatggtactcatttaatgcactggtaccaacagaaaccaggacagccacccaaactcctcatctatgctgcatccaacctagaatctggagtccctgccaggttcagtggcggtgggtctgagacagacttcaccctcaacatccatcctgtggaggaggaggatggtgcaacctatttctgtcagcaaagtattgagtatcctcggacgttcggtggaggcaccaagctggaaatcaatcgtacggtggccgcccccagcgtgttcatcttcccccccagcgatgagcagctgaagagcggcaccgccagcgtggtgtgtctgctgaacaacttctacccccgggaggccaaggtgcagtggaaggtggacaatgccctgcagagcggcaacagccaggagagcgtgaccgagcaggacagcaaggactccacctacagcctgagcagcaccctgaccctgagcaaggccgactacgagaagcacaaggtgtacgcctgtgaggtgacccaccagggcctgtccagccccgtgaccaagagcttcaaccggggcgagtgc

SEQ ID NO: 164 - protein, 5 aa, mus musculus
DYYNM

SEQ ID NO: 165 - protein, 16 aa, mus musculus
VINPYNGGTDYNQKFG

SEQ ID NO: 166 - protein, 9 aa, mus musculus
SVYDYPFDY

SEQ ID NO: 167 - protein, 15 aa, mus musculus
RASESVSIHGTHLMH

SEQ ID NO: 168 - protein, 7 aa, mus musculus
AASNLES

SEQ ID NO: 169 - protein, 9 aa, mus musculus
QQSIEDPRT

SEQ ID NO: 170 - protein, 5 aa, mus musculus
DYSID

SEQ ID NO: 171 - protein, 17 aa, mus musculus
DIDPNYGDPIYNHKFKG

SEQ ID NO: 172 - protein, 10 aa, mus musculus
RATGTDWFAF

SEQ ID NO: 173 - protein, 11 aa, mus musculus
RASENIYNNLA

SEQ ID NO: 174 - protein, 7 aa, mus musculus
AATILAD

SEQ ID NO: 175 - protein, 9 aa, mus musculus
QHFWGTPLT

SEQ ID NO: 176 - protein, 5 aa, mus musculus
NYWMH

SEQ ID NO: 177 - protein, 17 aa, mus musculus
IIHPNSGSTNYNEKFKS

SEQ ID NO: 178 - protein, 9 aa, mus musculus
GIYDYPFAY

SEQ ID NO: 179 - protein, 15 aa, mus musculus
RASESVSIHGTHLMH

SEQ ID NO: 180 - protein, 7 aa, mus musculus
AASNLES

SEQ ID NO: 181 - protein, 9 aa, mus musculus
QQSIEDPYT

SEQ ID NO: 182 - protein, 5 aa, mus musculus
RYWMS

SEQ ID NO: 183 - protein, 17 aa, mus musculus
EINPDRSTINYAPSLKD

SEQ ID NO: 184 - protein, 11 aa, mus musculus
FYYDYEGAMDY

SEQ ID NO: 185 - protein, 11 aa, mus musculus
KASQNVDTNVA

SEQ ID NO: 186 - protein, 7 aa, mus musculus
SASYRFS

SEQ ID NO: 187 - protein, 9 aa, mus musculus
QQYNSFPFT

SEQ ID NO: 188 - protein, 5 aa, mus musculus
SYWMH

SEQ ID NO: 189 - protein, 17 aa, mus musculus
VIDPSDSYTNYNQKFKG

SEQ ID NO: 190 - protein, 9 aa, mus musculus
QVFDYPMDY

SEQ ID NO: 191 - protein, 15 aa, mus musculus
RASESVSIHGTHLMH

SEQ ID NO: 192 - protein, 7 aa, mus musculus
AASNLES

SEQ ID NO: 193 - protein, 9 aa, mus musculus
QQSIEDPWT

SEQ ID NO: 194 - protein, 5 aa, mus musculus
DYEMH

SEQ ID NO: 195 - protein, 17 aa, mus musculus
AIDPETGGTAYNQKFKG

SEQ ID NO: 196 - protein, 9 aa, mus musculus
SIYDYYFDY

SEQ ID NO: 197 - protein, 15 aa, mus musculus
RASESVSIHGTHLMH

SEQ ID NO: 198 - protein, 7 aa, mus musculus
AASNLES

SEQ ID NO: 199 - protein, 9 aa, mus musculus
QQSIEYPRT